European Patent Application EP 4 130 273 A1, published February 8, 2023. Title: Production of Heterologous Polypeptides in Microalgae, Microalgal Extracellular Bodies, Compositions, and Methods of Making and Uses Thereof. Applicant: Sanofi Vaccine Technologies, S.A.S. Application To Be Assigned. The sequence listing filed with the application follows.

SEQUENCE LISTING (103 sequences)

SEQ ID NO: 1 - protein, 35 aa, Schizochytrium
MANIMANVTPQGVAKGFGLFVGVLFFLYWFLVGLA

SEQ ID NO: 2 - DNA, 105 bp, Schizochytrium
atggccaacatcatggccaacgtcacgccccagggcgtcgccaagggctttggcctctttgtcggcgtgctcttctttctctactggttccttgtcggcctcgcc

SEQ ID NO: 3 - DNA, 1999 bp, Schizochytrium
ccgcgaatcaagaaggtaggcgcgctgcgaggcgcggcggcggagcggagcgagggagagggagagggagagagagggagggagacgtcgccgcggcggggcctggcctggcctggtttggcttggtcagcgcggccttgtccgagcgtgcagctggagttgggtggattcatttggattttcttttgtttttgtttttctctctttcccggaaagtgttggccggtcggtgttctttgttttgatttcttcaaaagttttggtggttggttctctctcttggctctctgtcaggcggtccggtccacgccccggcctctcctctcctctcctctcctctcctctccgtgcgtatacgtacgtacgtttgtatacgtacatacatcccgcccgccgtgccggcgagggtttgctcagcctggagcaatgcgatgcgatgcgatgcgatgcgacgcgacgcgacgcgagtcactggttcgcgctgtggctgtggcttgcttgcttacttgctttcgagctctcccgctttcttctttccttctcacgccaccaccaacgaaagaagatcggccccggcacgccgctgagaagggctggcggcgatgacggcacgcgcgcccgctgccacgttggcgctcgctgctgctgctgctgctgctgctgctgctgctgctgctgctgctgctgcttctgcgcgcaggctttgccacgaggccggcgtgctggccgctgccgcttccagtccgcgtggagagatcgaatgagagataaactggatggattcatcgagggatgaatgaacgatggttggatgcctttttcctttttcaggtccacagcgggaagcaggagcgcgtgaatctgccgccatccgcatacgtctgcatcgcatcgcatcgcatgcacgcatcgctcgccgggagccacagacgggcgacagggcggccagccagccaggcagccagccaggcaggcaccagagggccagagagcgcgcctcacgcacgcgccgcagtgcgcgcatcgctcgcagtgcagaccttgattccccgcgcggatctccgcgagcccgaaacgaagagcgccgtacgggcccatcctagcgtcgcctcgcaccgcatcgcatcgcatcgcgttccctagagagtagtactcgacgaaggcaccatttccgcgctcctcttcggcgcgatcgaggcccccggcgccgcgacgatcgcggcggccgcggcgctggcggcggccctggcgctcgcgctggcggccgccgcgggcgtctggccctggcgcgcgcgggcgccgcaggaggagcggcagcggctgctcgccgccagagaaggagcgcgccgggcccggggagggacggggaggagaaggagaaggcgcgcaaggcggccccgaaagagaagaccctggacttgaacgcgaagaagaagaagaaggagaagaagttgaagaagaagaagaagaaggagaggaagttgaagaagacgaggagcaggcgcgttccaaggcgcgttctcttccggaggcgcgttccagctgcggcggcggggcgggctgcggggcgggcgcgggcgcgggtgcgggcagaggggacgcgcgcgcggaggcggagggggccgagcgggagcccctgctgctgcggggcgcccgggccgcaggtgtggcgcgcgcgacgacggaggcgacgacgccagcggccgcgacgacaaggccggcggcgtcggcgggcggaaggccccgcgcggagcaggggcgggagcaggacaaggcgcaggagcaggagcagggccgggagcgggagcgggagcgggcggcggagcccgaggcagaacccaatcgagatccagagcgagcagaggccggccgcgagcccgagcccgcgccgcagatcactagtaccgctgcggaatcacagcagcagcagcagcagcagcagcagcagcagcagcagcagcagccacgagagggagataaagaaaaagcggcagagacg

SEQ ID NO: 4 - DNA, 325 bp, Schizochytrium
gatccgaaagtgaaccttgtcctaacccgacagcgaatggcgggagggggcgggctaaaagatcgtattacatagtatttttcccctactctttgtgtttgtctttttttttttttgaacgcattcaagccacttgtcttggtttacttgtttgtttgcttgcttgcttgcttgcttgcctgcttcttggtcagacggcccaaaaaagggaaaaaattcattcatggcacagataagaaaaagaaaaagtttgtcgaccaccgtcatcagaaagcaagagaagagaaacactcgcgctcacattctcgctcgcgtaagaatctta

SEQ ID NO: 5 - DNA, 372 bp, Streptoalloteichus hindustanus
atggccaagttgaccagtgccgttccggtgctcaccgcgcgcgacgtcgccggagcggtcgagttctggaccgaccggctcgggttctcccgggacttcgtggaggacgacttcgccggtgtggtccgggacgacgtgaccctgttcatcagcgcggtccaggaccaggtggtgccggacaacaccctggcctgggtgtgggtgcgcggcctggacgagctgtacgccgagtggtcggaggtcgtgtccacgaacttccgggacgcctccgggccggccatgaccgagatcggcgagcagccgtgggggcgggagttcgccctgcgcgacccggccggcaactgcgtgcacttcgtggccgaggagcaggac

SEQ ID NO: 6 - DNA, 2055 bp, Schizochytrium
atgagcgcgacccgcgcggcgacgaggacagcggcggcgctgtcctcggcgctgacgacgcctgtaaagcagcagcagcagcagcagctgcgcgtaggcgcggcgtcggcacggctggcggccgcggcgttctcgtccggcacgggcggagacgcggccaagaaggcggccgcggcgagggcgttctccacgggacgcggccccaacgcgacacgcgagaagagctcgctggccacggtccaggcggcgacggacgatgcgcgcttcgtcggcctgaccggcgcccaaatctttcatgagctcatgcgcgagcaccaggtggacaccatctttggctaccctggcggcgccattctgcccgtttttgatgccatttttgagagtgacgccttcaagttcattctcgctcgccacgagcagggcgccggccacatggccgagggctacgcgcgcgccacgggcaagcccggcgttgtcctcgtcacctcgggccctggagccaccaacaccatcaccccgatcatggatgcttacatggacggtacgccgctgctcgtgttcaccggccaggtgcccacctctgctgtcggcacggacgctttccaggagtgtgacattgttggcatcagccgcgcgtgcaccaagtggaacgtcatggtcaaggacgtgaaggagctcccgcgccgcatcaatgaggcctttgagattgccatgagcggccgcccgggtcccgtgctcgtcgatcttcctaaggatgtgaccgccgttgagctcaaggaaatgcccgacagctccccccaggttgctgtgcgccagaagcaaaaggtcgagcttttccacaaggagcgcattggcgctcctggcacggccgacttcaagctcattgccgagatgatcaaccgtgcggagcgacccgtcatctatgctggccagggtgtcatgcagagcccgttgaatggcccggctgtgctcaaggagttcgcggagaaggccaacattcccgtgaccaccaccatgcagggtctcggcggctttgacgagcgtagtcccctctccctcaagatgctcggcatgcacggctctgcctacgccaactactcgatgcagaacgccgatcttatcctggcgctcggtgcccgctttgatgatcgtgtgacgggccgcgttgacgcctttgctccggaggctcgccgtgccgagcgcgagggccgcggtggcatcgttcactttgagatttcccccaagaacctccacaaggtcgtccagcccaccgtcgcggtcctcggcgacgtggtcgagaacctcgccaacgtcacgccccacgtgcagcgccaggagcgcgagccgtggtttgcgcagatcgccgattggaaggagaagcacccttttctgctcgagtctgttgattcggacgacaaggttctcaagccgcagcaggtcctcacggagcttaacaagcagattctcgagattcaggagaaggacgccgaccaggaggtctacatcaccacgggcgtcggaagccaccagatgcaggcagcgcagttccttacctggaccaagccgcgccagtggatctcctcgggtggcgccggcactatgggctacggccttccctcggccattggcgccaagattgccaagcccgatgctattgttattgacatcgatggtgatgcttcttattcgatgaccggtatggaattgatcacagcagccgaattcaaggttggcgtgaagattcttcttttgcagaacaactttcagggcatggtcaagaactggcaggatctcttttacgacaagcgctactcgggcaccgccatgttcaacccgcgcttcgacaaggtcgccgatgcgatgcgtgccaagggtctctactgcgcgaaacagtcggagctcaaggacaagatcaaggagtttctcgagtacgatgagggtcccgtcctcctcgaggttttcgtggacaaggacacgctcgtcttgcccatggtccccgctggctttccgctccacgagatggtcctcgagcctcctaagcccaaggacgcctaa

SEQ ID NO: 7 - protein, 684 aa, Schizochytrium
MSATRAATRTAAALSSALTTPVKQQQQQQLRVGAASARLAAAAFSSGTGGDAAKKAAAARAFSTGRGPNATREKSSLATVQAATDDARFVGLTGAQIFHELMREHQVDTIFGYPGGAILPVFDAIFESDAFKFILARHEQGAGHMAEGYARATGKPGVVLVTSGPGATNTITPIMDAYMDGTPLLVFTGQVPTSAVGTDAFQECDIVGISRACTKWNVMVKDVKELPRRINEAFEIAMSGRPGPVLVDLPKDVTAVELKEMPDSSPQVAVRQKQKVELFHKERIGAPGTADFKLIAEMINRAERPVIYAGQGVMQSPLNGPAVLKEFAEKANIPVTTTMQGLGGFDERSPLSLKMLGMHGSAYANYSMQNADLILALGARFDDRVTGRVDAFAPEARRAEREGRGGIVHFEISPKNLHKVVQPTVAVLGDVVENLANVTPHVQRQEREPWFAQIADWKEKHPFLLESVDSDDKVLKPQQVLTELNKQILEIQEKDADQEVYITTGVGSHQMQAAQFLTWTKPRQWISSGGAGTMGYGLPSAIGAKIAKPDAIVIDIDGDASYSMTGMELITAAEFKVGVKILLLQNNFQGMVKNWQDLFYDKRYSGTAMFNPRFDKVADAMRAKGLYCAKQSELKDKIKEFLEYDEGPVLLEVFVDKDTLVLPMVPAGFPLHEMVLEPPKPKDA

SEQ ID NO: 8 - protein, 684 aa, Artificial Sequence
  Mutated ALS 1
MSATRAATRTAAALSSALTTPVKQQQQQQLRVGAASARLAAAAFSSGTGGDAAKKAAAARAFSTGRGPNATREKSSLATVQAATDDARFVGLTGAQIFHELMREHQVDTIFGYPGGAILPVFDAIFESDAFKFILARHEQGAGHMAEGYARATGKPGVVLVTSGPGATNTITPIMDAYMDGTPLLVFTGQVPTSAVGTDAFQECDIVGISRACTKWNVMVKDVKELPRRINEAFEIAMSGRPGPVLVDLPKDVTAVELKEMPDSSPQVAVRQKQKVELFHKERIGAPGTADFKLIAEMINRAERPVIYAGQGVMQSPLNGPAVLKEFAEKANIPVTTTMQGLGGFDERSPLSLKMLGMHGSAYANYSMQNADLILALGARFDDRVTGRVDAFAPEARRAEREGRGGIVHFEISPKNLHKVVQPTVAVLGDVVENLANVTPHVQRQEREPWFAQIADWKEKHPFLLESVDSDDKVLKPQQVLTELNKQILEIQEKDADQEVYITTGVGSHQMQAAQFLTWTKPRQWISSGGAGTMGYGLPSAIGAKIAKPDAIVIDIDGDASYSMTGMELITAAEFKVGVKILLLQNNFQGMVKNVQDLFYDKRYSGTAMFNPRFDKVADAMRAKGLYCAKQSELKDKIKEFLEYDEGPVLLEVFVDKDTLVLPMVPAGFPLHEMVLEPPKPKDA

SEQ ID NO: 9 - protein, 684 aa, Artificial Sequence
  Mutated ALS 2
MSATRAATRTAAALSSALTTPVKQQQQQQLRVGAASARLAAAAFSSGTGGDAAKKAAAARAFSTGRGPNATREKSSLATVQAATDDARFVGLTGAQIFHELMREHQVDTIFGYPGGAILPVFDAIFESDAFKFILARHEQGAGHMAEGYARATGKPGVVLVTSGPGATNTITPIMDAYMDGTPLLVFTGQVQTSAVGTDAFQECDIVGISRACTKWNVMVKDVKELPRRINEAFEIAMSGRPGPVLVDLPKDVTAVELKEMPDSSPQVAVRQKQKVELFHKERIGAPGTADFKLIAEMINRAERPVIYAGQGVMQSPLNGPAVLKEFAEKANIPVTTTMQGLGGFDERSPLSLKMLGMHGSAYANYSMQNADLILALGARFDDRVTGRVDAFAPEARRAEREGRGGIVHFEISPKNLHKVVQPTVAVLGDVVENLANVTPHVQRQEREPWFAQIADWKEKHPFLLESVDSDDKVLKPQQVLTELNKQILEIQEKDADQEVYITTGVGSHQMQAAQFLTWTKPRQWISSGGAGTMGYGLPSAIGAKIAKPDAIVIDIDGDASYSMTGMELITAAEFKVGVKILLLQNNFQGMVKNWQDLFYDKRYSGTAMFNPRFDKVADAMRAKGLYCAKQSELKDKIKEFLEYDEGPVLLEVFVDKDTLVLPMVPAGFPLHEMVLEPPKPKDA

SEQ ID NO: 10 - protein, 684 aa, Artificial Sequence
  Mutated ALS 3
MSATRAATRTAAALSSALTTPVKQQQQQQLRVGAASARLAAAAFSSGTGGDAAKKAAAARAFSTGRGPNATREKSSLATVQAATDDARFVGLTGAQIFHELMREHQVDTIFGYPGGAILPVFDAIFESDAFKFILARHEQGAGHMAEGYARATGKPGVVLVTSGPGATNTITPIMDAYMDGTPLLVFTGQVQTSAVGTDAFQECDIVGISRACTKWNVMVKDVKELPRRINEAFEIAMSGRPGPVLVDLPKDVTAVELKEMPDSSPQVAVRQKQKVELFHKERIGAPGTADFKLIAEMINRAERPVIYAGQGVMQSPLNGPAVLKEFAEKANIPVTTTMQGLGGFDERSPLSLKMLGMHGSAYANYSMQNADLILALGARFDDRVTGRVDAFAPEARRAEREGRGGIVHFEISPKNLHKVVQPTVAVLGDVVENLANVTPHVQRQEREPWFAQIADWKEKHPFLLESVDSDDKVLKPQQVLTELNKQILEIQEKDADQEVYITTGVGSHQMQAAQFLTWTKPRQWISSGGAGTMGYGLPSAIGAKIAKPDAIVIDIDGDASYSMTGMELITAAEFKVGVKILLLQNNFQGMVKNVQDLFYDKRYSGTAMFNPRFDKVADAMRAKGLYCAKQSELKDKIKEFLEYDEGPVLLEVFVDKDTLVLPMVPAGFPLHEMVLEPPKPKDA

SEQ ID NO: 11 - DNA, 2052 bp, Artificial Sequence
  Mutated ALS 1
atgagcgcgacccgcgcggcgacgaggacagcggcggcgctgtcctcggcgctgacgacgcctgtaaagcagcagcagcagcagcagctgcgcgtaggcgcggcgtcggcacggctggcggccgcggcgttctcgtccggcacgggcggagacgcggccaagaaggcggccgcggcgagggcgttctccacgggacgcggccccaacgcgacacgcgagaagagctcgctggccacggtccaggcggcgacggacgatgcgcgcttcgtcggcctgaccggcgcccaaatctttcatgagctcatgcgcgagcaccaggtggacaccatctttggctaccctggcggcgccattctgcccgtttttgatgccatttttgagagtgacgccttcaagttcattctcgctcgccacgagcagggcgccggccacatggccgagggctacgcgcgcgccacgggcaagcccggcgttgtcctcgtcacctcgggccctggagccaccaacaccatcaccccgatcatggatgcttacatggacggtacgccgctgctcgtgttcaccggccaggtgcccacctctgctgtcggcacggacgctttccaggagtgtgacattgttggcatcagccgcgcgtgcaccaagtggaacgtcatggtcaaggacgtgaaggagctcccgcgccgcatcaatgaggcctttgagattgccatgagcggccgcccgggtcccgtgctcgtcgatcttcctaaggatgtgaccgccgttgagctcaaggaaatgcccgacagctccccccaggttgctgtgcgccagaagcaaaaggtcgagcttttccacaaggagcgcattggcgctcctggcacggccgacttcaagctcattgccgagatgatcaaccgtgcggagcgacccgtcatctatgctggccagggtgtcatgcagagcccgttgaatggcccggctgtgctcaaggagttcgcggagaaggccaacattcccgtgaccaccaccatgcagggtctcggcggctttgacgagcgtagtcccctctccctcaagatgctcggcatgcacggctctgcctacgccaactactcgatgcagaacgccgatcttatcctggcgctcggtgcccgctttgatgatcgtgtgacgggccgcgttgacgcctttgctccggaggctcgccgtgccgagcgcgagggccgcggtggcatcgttcactttgagatttcccccaagaacctccacaaggtcgtccagcccaccgtcgcggtcctcggcgacgtggtcgagaacctcgccaacgtcacgccccacgtgcagcgccaggagcgcgagccgtggtttgcgcagatcgccgattggaaggagaagcacccttttctgctcgagtctgttgattcggacgacaaggttctcaagccgcagcaggtcctcacggagcttaacaagcagattctcgagattcaggagaaggacgccgaccaggaggtctacatcaccacgggcgtcggaagccaccagatgcaggcagcgcagttccttacctggaccaagccgcgccagtggatctcctcgggtggcgccggcactatgggctacggccttccctcggccattggcgccaagattgccaagcccgatgctattgttattgacatcgatggtgatgcttcttattcgatgaccggtatggaattgatcacagcagccgaattcaaggttggcgtgaagattcttcttttgcagaacaactttcagggcatggtcaagaacgttcaggatctcttttacgacaagcgctactcgggcaccgccatgttcaacccgcgcttcgacaaggtcgccgatgcgatgcgtgccaagggtctctactgcgcgaaacagtcggagctcaaggacaagatcaaggagtttctcgagtacgatgagggtcccgtcctcctcgaggttttcgtggacaaggacacgctcgtcttgcccatggtccccgctggctttccgctccacgagatggtcctcgagcctcctaagcccaaggacgcc

SEQ ID NO: 12 - DNA, 2052 bp, Artificial Sequence
  Mutated ALS 2
atgagcgcgacccgcgcggcgacgaggacagcggcggcgctgtcctcggcgctgacgacgcctgtaaagcagcagcagcagcagcagctgcgcgtaggcgcggcgtcggcacggctggcggccgcggcgttctcgtccggcacgggcggagacgcggccaagaaggcggccgcggcgagggcgttctccacgggacgcggccccaacgcgacacgcgagaagagctcgctggccacggtccaggcggcgacggacgatgcgcgcttcgtcggcctgaccggcgcccaaatctttcatgagctcatgcgcgagcaccaggtggacaccatctttggctaccctggcggcgccattctgcccgtttttgatgccatttttgagagtgacgccttcaagttcattctcgctcgccacgagcagggcgccggccacatggccgagggctacgcgcgcgccacgggcaagcccggcgttgtcctcgtcacctcgggccctggagccaccaacaccatcaccccgatcatggatgcttacatggacggtacgccgctgctcgtgttcaccggccaggtgcagacctctgctgtcggcacggacgctttccaggagtgtgacattgttggcatcagccgcgcgtgcaccaagtggaacgtcatggtcaaggacgtgaaggagctcccgcgccgcatcaatgaggcctttgagattgccatgagcggccgcccgggtcccgtgctcgtcgatcttcctaaggatgtgaccgccgttgagctcaaggaaatgcccgacagctccccccaggttgctgtgcgccagaagcaaaaggtcgagcttttccacaaggagcgcattggcgctcctggcacggccgacttcaagctcattgccgagatgatcaaccgtgcggagcgacccgtcatctatgctggccagggtgtcatgcagagcccgttgaatggcccggctgtgctcaaggagttcgcggagaaggccaacattcccgtgaccaccaccatgcagggtctcggcggctttgacgagcgtagtcccctctccctcaagatgctcggcatgcacggctctgcctacgccaactactcgatgcagaacgccgatcttatcctggcgctcggtgcccgctttgatgatcgtgtgacgggccgcgttgacgcctttgctccggaggctcgccgtgccgagcgcgagggccgcggtggcatcgttcactttgagatttcccccaagaacctccacaaggtcgtccagcccaccgtcgcggtcctcggcgacgtggtcgagaacctcgccaacgtcacgccccacgtgcagcgccaggagcgcgagccgtggtttgcgcagatcgccgattggaaggagaagcacccttttctgctcgagtctgttgattcggacgacaaggttctcaagccgcagcaggtcctcacggagcttaacaagcagattctcgagattcaggagaaggacgccgaccaggaggtctacatcaccacgggcgtcggaagccaccagatgcaggcagcgcagttccttacctggaccaagccgcgccagtggatctcctcgggtggcgccggcactatgggctacggccttccctcggccattggcgccaagattgccaagcccgatgctattgttattgacatcgatggtgatgcttcttattcgatgaccggtatggaattgatcacagcagccgaattcaaggttggcgtgaagattcttcttttgcagaacaactttcagggcatggtcaagaactggcaggatctcttttacgacaagcgctactcgggcaccgccatgttcaacccgcgcttcgacaaggtcgccgatgcgatgcgtgccaagggtctctactgcgcgaaacagtcggagctcaaggacaagatcaaggagtttctcgagtacgatgagggtcccgtcctcctcgaggttttcgtggacaaggacacgctcgtcttgcccatggtccccgctggctttccgctccacgagatggtcctcgagcctcctaagcccaaggacgcc

SEQ ID NO: 13 - DNA, 2055 bp, Artificial Sequence
  Mutated ALS 3
atgagcgcgacccgcgcggcgacgaggacagcggcggcgctgtcctcggcgctgacgacgcctgtaaagcagcagcagcagcagcagctgcgcgtaggcgcggcgtcggcacggctggcggccgcggcgttctcgtccggcacgggcggagacgcggccaagaaggcggccgcggcgagggcgttctccacgggacgcggccccaacgcgacacgcgagaagagctcgctggccacggtccaggcggcgacggacgatgcgcgcttcgtcggcctgaccggcgcccaaatctttcatgagctcatgcgcgagcaccaggtggacaccatctttggctaccctggcggcgccattctgcccgtttttgatgccatttttgagagtgacgccttcaagttcattctcgctcgccacgagcagggcgccggccacatggccgagggctacgcgcgcgccacgggcaagcccggcgttgtcctcgtcacctcgggccctggagccaccaacaccatcaccccgatcatggatgcttacatggacggtacgccgctgctcgtgttcaccggccaggtgcagacctctgctgtcggcacggacgctttccaggagtgtgacattgttggcatcagccgcgcgtgcaccaagtggaacgtcatggtcaaggacgtgaaggagctcccgcgccgcatcaatgaggcctttgagattgccatgagcggccgcccgggtcccgtgctcgtcgatcttcctaaggatgtgaccgccgttgagctcaaggaaatgcccgacagctccccccaggttgctgtgcgccagaagcaaaaggtcgagcttttccacaaggagcgcattggcgctcctggcacggccgacttcaagctcattgccgagatgatcaaccgtgcggagcgacccgtcatctatgctggccagggtgtcatgcagagcccgttgaatggcccggctgtgctcaaggagttcgcggagaaggccaacattcccgtgaccaccaccatgcagggtctcggcggctttgacgagcgtagtcccctctccctcaagatgctcggcatgcacggctctgcctacgccaactactcgatgcagaacgccgatcttatcctggcgctcggtgcccgctttgatgatcgtgtgacgggccgcgttgacgcctttgctccggaggctcgccgtgccgagcgcgagggccgcggtggcatcgttcactttgagatttcccccaagaacctccacaaggtcgtccagcccaccgtcgcggtcctcggcgacgtggtcgagaacctcgccaacgtcacgccccacgtgcagcgccaggagcgcgagccgtggtttgcgcagatcgccgattggaaggagaagcacccttttctgctcgagtctgttgattcggacgacaaggttctcaagccgcagcaggtcctcacggagcttaacaagcagattctcgagattcaggagaaggacgccgaccaggaggtctacatcaccacgggcgtcggaagccaccagatgcaggcagcgcagttccttacctggaccaagccgcgccagtggatctcctcgggtggcgccggcactatgggctacggccttccctcggccattggcgccaagattgccaagcccgatgctattgttattgacatcgatggtgatgcttcttattcgatgaccggtatggaattgatcacagcagccgaattcaaggttggcgtgaagattcttcttttgcagaacaactttcagggcatggtcaagaacgttcaggatctcttttacgacaagcgctactcgggcaccgccatgttcaacccgcgcttcgacaaggtcgccgatgcgatgcgtgccaagggtctctactgcgcgaaacagtcggagctcaaggacaagatcaaggagtttctcgagtacgatgagggtcccgtcctcctcgaggttttcgtggacaaggacacgctcgtcttgcccatggtccccgctggctttccgctccacgagatggtcctcgagcctcctaagcccaaggacgcctaa

SEQ ID NO: 14 - DNA, 12 bp, Schizochytrium
cacgacgagttg

SEQ ID NO: 15 - protein, 53 aa, Schizochytrium
MANIMANVTPQGVAKGFGLFVGVLFFLYWFLVGLALLGDGFKVIAGDSAGTLF

SEQ ID NO: 16 - DNA, 21 bp, Artificial Sequence
  Synthetic Primer S4termF
gatcccatggcacgtgctacg

SEQ ID NO: 17 - DNA, 22 bp, Artificial Sequence
  Synthetic Primer S4termR
ggcaacatgtatgataagatac

SEQ ID NO: 18 - DNA, 21 bp, Artificial Sequence
  Synthetic Primer C2mcsSmaF
gatccccgggttaagcttggt

SEQ ID NO: 19 - DNA, 20 bp, Artificial Sequence
  Synthetic Primer C2mcsSmaR
actggggcccgtttaaactc

SEQ ID NO: 20 - DNA, 34 bp, Artificial Sequence
  Synthetic Primer 5'tubMCS_BglI
gactagatctcaattttaggccccccactgaccg

SEQ ID NO: 21 - DNA, 34 bp, Artificial Sequence
  Synthetic Primer 3'SV40MCS_Sal
gactgtcgaccatgtatgataagatacattgatg

SEQ ID NO: 22 - DNA, 28 bp, Artificial Sequence
  Synthetic Primer 5'ALSproNde3
gactcatatggcccaggcctactttcac

SEQ ID NO: 23 - DNA, 34 bp, Artificial Sequence
  Synthetic Primer 3'ALStermBglII
gactagatctgggtcaaggcagaagaattccgcc

SEQ ID NO: 24 - DNA, 97 bp, Artificial Sequence
  Synthetic Primer sec.Gfp5'1b
tactggttccttgtcggcctcgcccttctcggcgatggcttcaaggtcatcgccggtgactccgccggtacgctcttcatggtgagcaagggcgagg

SEQ ID NO: 25 - DNA, 32 bp, Artificial Sequence
  Synthetic Primer sec.Gfp3'Spe
gatcggtaccggtgttctttgttttgatttct

SEQ ID NO: 26 - DNA, 105 bp, Artificial Sequence
  Synthetic Primer sec.Gfp5'Bam
taatggatccatggccaacatcatggccaacgtcacgccccagggcgtcgccaagggctttggcctctttgtcggcgtgctcttctttctctactggttccttgt

SEQ ID NO: 27 - DNA, 40 bp, Artificial Sequence
  Synthetic Primer ss.eGfpHELD3'RV
cctgatatcttacaactcgtcgtggttgtacagctcgtcc

SEQ ID NO: 28 - DNA, 105 bp, Artificial Sequence; identical to SEQ ID NO: 26
  Synthetic Primer sec.Gfp5'Bam2

SEQ ID NO: 29 - DNA, 27 bp, Artificial Sequence
  Synthetic Primer prREZ15
cggtacccgcgaatcaagaaggtaggc

SEQ ID NO: 30 - DNA, 27 bp, Artificial Sequence
  Synthetic Primer prREZ16
cggatcccgtctctgccgctttttctt

SEQ ID NO: 31 - DNA, 30 bp, Artificial Sequence
  Synthetic Primer prREZ17
cggatccgaaagtgaaccttgtcctaaccc

SEQ ID NO: 32 - DNA, 27 bp, Artificial Sequence
  Synthetic Primer prREZ18
ctctagacagatccgcaccatcggccg

SEQ ID NO: 33 - DNA, 32 bp, Artificial Sequence
  Synthetic Primer 5'eGFP_kpn
gactggtaccatggtgaagcaagggcgaggag

SEQ ID NO: 34 - DNA, 34 bp, Artificial Sequence
  Synthetic Primer 3'eGFP_xba
gacttctagattacttgtacagctcgtccatgcc

SEQ ID NO: 35 - DNA, 32 bp, Artificial Sequence; identical to SEQ ID NO: 25
  Synthetic Primer 5'ORFCproKpn-2

SEQ ID NO: 36 - DNA, 31 bp, Artificial Sequence
  Synthetic Primer 3'ORFCproKpn-2
gatcggtaccgtctctgccgctttttcttta

SEQ ID NO: 37 - protein, 20 aa, Schizochytrium
MKFATSVAILLVANIATALA

SEQ ID NO: 38 - DNA, 60 bp, Schizochytrium
atgaagttcgcgacctcggtcgcaattttgcttgtggccaacatagccaccgccctcgcg

SEQ ID NO: 39 - DNA, 28 bp, Artificial Sequence
  Synthetic Primer 5'ss-X Bgl long
gactagatctatgaagttcgcgacctcg

SEQ ID NO: 40 - DNA, 33 bp, Artificial Sequence
  Synthetic Primer 3'ritx_kap_bh_Bgl
gactagatcttcagcactcaccgcggttaaagg

SEQ ID NO: 41 - DNA, 702 bp, Artificial Sequence
  Optimized Sec1
atgaagttcgcgacctcggtcgcaattttgcttgtggccaacatagccaccgccctcgcgcagatcgtcctcagccagtcccccgccatcctttccgcttcccccggtgagaaggtgaccatgacctgccgcgctagctcctccgtctcgtacatccactggttccagcagaagcccggctcgtcccccaagccctggatctacgccacctccaacctcgcctccggtgttcccgttcgtttttccggttccggttccggcacctcctactccctcaccatctcccgcgtcgaggccgaggatgccgccacctactactgccagcagtggaccagcaacccccccaccttcggcggtggtacgaagctcgagattaagcgcaccgtcgccgccccctccgtcttcatttttcccccctccgatgagcagctcaagtccggtaccgcctccgtcgtttgcctcctcaacaacttctacccccgtgaggccaaggtccagtggaaggtcgacaacgcgcttcagtccggtaactcccaggagtccgtcaccgagcaggattcgaaggacagcacctactccctctcctccaccctcaccctctccaaggccgactacgagaagcacaaggtctacgcctgcgaggtcacgcaccagggtctttcctcccccgtcacgaagtcctttaaccgcggtgagtgctga

SEQ ID NO: 42 - DNA, 853 bp, Schizochytrium
ctccatcgatcgtgcggtcaaaaagaaaggaagaagaaaggaaaaagaaaggcgtgcgcacccgagtgcgcgctgagcgcccgctcgcggccccgcggagcctccgcgttagtccccgccccgcgccgcgcagtcccccgggaggcatcgcgcacctctcgccgccccctcgcgcctcgccgattccccgcctccccttttccgcttcttcgccgcctccgctcgcggccgcgtcgcccgcgccccgctccctatctgctccccaggggggcactccgcaccttttgcgcccgctgccgccgccgcggccgccccgccgccctggtttcccccgcgagcgcggccgcgtcgccgcgcaaagactcgccgcgtgccgccccgagcaacgggtggcggcggcgcggcggcgggcggggcgcggcggcgcgtaggcggggctaggcgccggctaggcgaaacgccgcccccgggcgccgccgccgcccgctccagagcagtcgccgcgccagaccgccaacgcagagaccgagaccgaggtacgtcgcgcccgagcacgccgcgacgcgcggcagggacgaggagcacgacgccgcgccgcgccgcgcggggggggggagggagaggcaggacgcgggagcgagcgtgcatgtttccgcgcgagacgacgccgcgcgcgctggagaggagataaggcgcttggatcgcgagagggccagccaggctggaggcgaaaatgggtggagaggatagtatcttgcgtgcttggacgaggagactgacgaggaggacggatacgtcgatgatgatgtgcacagagaagaagcagttcgaaagcgactactagcaagcaagg

SEQ ID NO: 43 - DNA, 1064 bp, Schizochytrium
ctcttatctgcctcgcgccgttgaccgccgcttgactcttggcgcttgccgctcgcatcctgcctcgctcgcgcaggcgggcgggcgagtgggtgggtccgcagccttccgcgctcgcccgctagctcgctcgcgccgtgctgcagccagcagggcagcaccgcacggcaggcaggtcccggcgcggatcgatcgatccatcgatccatcgatccatcgatcgtgcggtcaaaaagaaaggaagaagaaaggaaaaagaaaggcgtgcgcacccgagtgcgcgctgagcgcccgctcgcggtcccgcggagcctccgcgttagtccccgccccgcgccgcgcagtcccccgggaggcatcgcgcacctctcgccgccccctcgcgcctcgccgattccccgcctccccttttccgcttcttcgccgcctccgctcgcggccgcgtcgcccgcgccccgctccctatctgctccccaggggggcactccgcaccttttgcgcccgctgccgccgccgcggccgccccgccgccctggtttcccccgcgagcgcggccgcgtcgccgcgcaaagactcgccgcgtgccgccccgagcaacgggtggcggcggcgcggcggcgggcggggcgcggcggcgcgtaggcggggctaggcgccggctaggcgaaacgccgcccccgggcgccgccgccgcccgctccagagcagtcgccgcgccagaccgccaacgcagagaccgagaccgaggtacgtcgcgcccgagcacgccgcgacgcgcggcagggacgaggagcacgacgccgcgccgcgccgcgcggggggggggagggagaggcaggacgcgggagcgagcgtgcatgtttccgcgcgagacgacgccgcgcgcgctggagaggagataaggcgcttggatcgcgagagggccagccaggctggaggcgaaaatgggtggagaggatagtatcttgcgtgcttggacgaggagactgacgaggaggacggatacgtcgatgatgatgtgcacagagaagaagcagttcgaaagcgactactagcaagcaagg

SEQ ID NO: 44 - DNA, 837 bp, Schizochytrium
cttcgctttctcaacctatctggacagcaatccgccacttgccttgatccccttccgcgcctcaatcactcgctccacgtccctcttccccctcctcatctccgtgctttctctgccccccccccccccgccgcggcgtgcgcgcgcgtggcgccgcggccgcgacaccttccatactatcctcgctcccaaaatgggttgcgctatagggcccggctaggcgaaagtctagcaggcacttgcttggcgcagagccgccgcggccgctcgttgccgcggatggagagggagagagagcccgcctcgataagcagagacagacagtgcgactgacagacagacagagagactggcagaccggaatacctcgaggtgagtgcggcgcgggcgagcgggcgggagcgggagcgcaagagggacggcgcggcgcggcggccctgcgcgacgccgcggcgtattctcgtgcgcagcgccgagcagcgggacgggcggctggctgatggttgaagcggggcggggtgaaatgttagatgagatgatcatcgacgacggtccgtgcgtcttggctggcttggctggcttggctggcgggcctgccgtgtttgcgagaaagaggatgaggagagcgacgaggaaggacgagaagactgacgtgtagggcgcgcgatggatgatcgattgattgattgattgattggttgattggctgtgtggtcgatgaacgtgtagactcagggagcgtggttaaattgttcttgcgccagacgcgaggactccacccccttctttcgcctttacacagcctttttgtgaagcaacaagaaagaaaaagccaag

SEQ ID NO: 45 - DNA, 1020 bp, Schizochytrium
ctttttccgctctgcataatcctaaaagaaagactataccctagtcactgtacaaatgggacatttctctcccgagcgatagctaaggatttttgcttcgtgtgcactgtgtgctctggccgcgcatcgaaagtccaggatcttactgtttctctttcctttcctttatttcctgttctcttcttcgctttctcaacctatctggacagcaatccgccacttgccttgatccccttccgcgcctcaatcactcgctccacgtccctcttccccctcctcatctccgtgctttctctcgccccccccccccccgccgcggcgtgcgcgcgcgtggcgccgcggccgcgacaccttccatactatcctcgctcccaaaatgggttgcgctatagggcccggctaggcgaaagtctagcaggcacttgcttggcgcagagccgccgcggccgctcgttgccgcggatggagagggagagagagcccgcctcgataagcagagacagacagtgcgactgacagacagacagagagactggcagaccggaatacctcgaggtgagtgcggcgcgggcgagcgggcgggagcgggagcgcaagagggacggcgcggcgcggcggccctgcgcgacgccgcggcgtattctcgtgcgcagcgccgagcagcgggacgggcggctggctgatggttgaagcggggcggggtgaaatgttagatgagatgatcatcgacgacggtccgtgcgtcttggctggcttggctggcttggctggcgggcctgccgtgtttgcgagaaagaggatgaggagagcgacgaggaaggacgagaagactgacgtgtagggcgcgcgatggatgatcgattgattgattgattgattggttgattggctgtgtggtcgatgaacgtgtagactcagggagcgtggttaaattgttcttgcgccagacgcgaggactccacccccttctttcgcctttacacagcctttttgtgaagcaacaagaaagaaaaagccaag

SEQ ID NO: 46 - DNA, 1416 bp, Schizochytrium
cccgtccttgacgccttcgcttccggcgcggccatcgattcaattcacccatccgatacgttccgccccctcacgtccgtctgcgcacgacccctgcacgaccacgccaaggccaacgcgccgctcagctcagcttgtcgacgagtcgcacgtcacatatctcagatgcattgcctgcctgcctgcctgcctgcctgcctgcctgcctgcctgcctgcctcagcctctctttgctctctctgcggcggccgctgcgacgcgctgtacaggagaatgactccaggaagtgcggctgggatacgcgctggcgtcggccgtgatgcgcgtgacgggcggcgggcacggccggcacgggttgagcagaggacgaagcgaggcgagacgagacaggccaggcgcggggagcgctcgctgccgtgagcagcagaccagggcgcaggaatgtacttttcttgcgggagcggagacgaggctgccggctgctggctgccggttgctctgcacgcgccgcccgacttggcgtagcgtggacgcgcggcggcggccgccgtctcgtcgcggtcggctttgccgtgtatcgacgctgcgggcttgacacgggatggcggaagttcagcatcgctgcgatccctcgcgccgcagaacgaggagagcgcaggccggcttcaagtttgaaaggagaggaaggcaggcaaggagctggaagcttgccgcggaaggcgcaggcatgcgtcacgtgaaaaaaagggatttcaagagtagtaagtaggtatggtctacaagtcccctattcttacttcgcggaacgtgggctgctcgtgcgggcgtccatcttgtttttgtttttttttccgctaggcgcgtgcattgcttgatgagtctcagcgttcgtctgcagcgagggcaggaaaataagcggcccgtgccgtcgagcgcacaggacgtgcaagcgccttgcgagcgcagcatccttgcacggcgagcatagagaccgcggccgatggactccagcgaggaattttcgaccctctctatcaagctgcgcttgacagccgggaatggcagcctgaggagagaggggcgaaggaagggacttggagaaaagaggtaaggcaccctcaatcacggcgcgtgaaagccagtcatccctcgcaaagaaaagacaaaagcgggttttttgtttcgatgggaaagaatttcttagaggaagaagcggcacacagactcgcgccatgcagatttctgcgcagctcgcgatcaaaccaggaacgtggtcgctgcgcgccactatcaggggtagcgcacgaataccaaacgcattactagctacgcgcctgtgacccgaggatcgggccacagacgttgtctcttgccatcccacgacctggcagcgagaagatcgtccattactcatcg

SEQ ID NO: 47 - DNA, 24 bp, Artificial Sequence
  Synthetic Primer 5'60S-807
tcgatttgcggatacttgctcaca

SEQ ID NO: 48 - DNA, 21 bp, Artificial Sequence
  Synthetic Primer 3'60S-2821
gacgacctcgcccttggacac

SEQ ID NO: 49 - DNA, 34 bp, Artificial Sequence
  Synthetic Primer 5'60Sp-1302-Kpn
gactggtacctttttccgctctgcataatcctaa

SEQ ID NO: 50 - DNA, 32 bp, Artificial Sequence
  Synthetic Primer 3'60Sp-Bam
gactggatccttggctttttctttcttgttgc

SEQ ID NO: 51 - DNA, 24 bp, Artificial Sequence
  Synthetic Primer 5'EF1-68
cgccgttgaccgccgcttgactct

SEQ ID NO: 52 - DNA, 24 bp, Artificial Sequence
  Synthetic Primer 3'EF1-2312
cgggggtagcctcggggatggact

SEQ ID NO: 53 - DNA, 34 bp, Artificial Sequence
  Synthetic Primer 5'EF1-54-Kpn
gactggtacctcttatctgcctcgcgccgttgac

SEQ ID NO: 54 - DNA, 37 bp, Artificial Sequence
  Synthetic Primer 5'EF1-1114-Bam
gactggatcccttgcttgctagtagtcgctttcgaac

SEQ ID NO: 55 - DNA, 29 bp, Artificial Sequence
  Synthetic Primer 5'Sec1P-kpn
gactggtaccccgtccttgacgccttcgc

SEQ ID NO: 56 - DNA, 31 bp, Artificial Sequence
  Synthetic Primer 3'Sec1P-ba
gactggatccgatgagtaatggacgatcttc

SEQ ID NO: 57 - DNA, 1614 bp, Artificial sequence
  Secretion signal
ggatccatgaagttcgcgacctcggtcgcaattttgcttgtggccaacatagccaccgccctcgcgtcgatgaccaacgagacctcggaccgccctctcgtgcactttacccccaacaagggttggatgaacgatcccaacggcctctggtacgacgagaaggatgctaagtggcacctttactttcagtacaaccctaacgacaccgtctggggcaccccgctcttctggggccacgccacctccgacgacctcaccaactgggaggaccagcccattgctatcgcccccaagcgcaacgactcgggagctttttccggttccatggttgtggactacaacaacacctccggtttttttaacgacaccattgacccccgccagcgctgcgtcgccatctggacctacaacacgcccgagagcgaggagcagtacatcagctacagccttgatggaggctacacctttaccgagtaccagaagaaccctgtcctcgccgccaactccacccagttccgcgaccctaaggttttttggtacgagccttcccagaagtggattatgaccgccgctaagtcgcaggattacaagatcgagatctacagcagcgacgacctcaagtcctggaagcttgagtccgcctttgccaacgagggttttctcggataccagtacgagtgccccggtctcatcgaggtccccaccgagcaggacccgtccaagtcctactgggtcatgtttatttccatcaaccctggcgcccctgccggcggcagcttcaaccagtacttcgtcggctcctttaacggcacgcattttgaggccttcgacaaccagtcccgcgtcgtcgacttcggcaaggactactacgccctccagaccttctttaacaccgaccccacctacggcagcgccctcggtattgcttgggcctccaactgggagtactccgctttcgtccccactaacccctggcgcagctcgatgtccctcgtccgcaagttttcgcttaacaccgagtaccaggccaaccccgagaccgagcttattaacctgaaggccgagcctattctcaacatctccaacgctggcccctggtcccgctttgctactaacactaccctcaccaaggccaactcctacaacgtcgatctctccaactccaccggtactcttgagtttgagctcgtctacgccgtcaacaccacccagaccatctccaagtccgtcttcgccgacctctccctctggttcaagggccttgaggaccccgaggagtacctgcgcatgggttttgaggtctccgcctcctccttcttcctcgatcgcggtaactccaaggttaagtttgtcaaggagaacccctactttactaaccgtatgagcgtcaacaaccagccctttaagtccgagaacgatcttagctactacaaggtttacggcctcctcgaccagaacattctcgagctctactttaacgacggagatgtcgtcagcaccaacacctactttatgaccactggaaacgccctcggcagcgtgaacatgaccaccggagtcgacaacctcttttacattgacaagtttcaggttcgcgaggttaagtaacatatg

SEQ ID NO: 58 - DNA, 11495 bp, Artificial sequence
  pCL0076
ctcttatctgcctcgcgccgttgaccgccgcttgactcttggcgcttgccgctcgcatcctgcctcgctcgcgcaggcgggcgggcgagtgggtgggtccgcagccttccgcgctcgcccgctagctcgctcgcgccgtgctgcagccagcagggcagcaccgcacggcaggcaggtcccggcgcggatcgatcgatccatcgatccatcgatccatcgatcgtgcggtcaaaaagaaaggaagaagaaaggaaaaagaaaggcgtgcgcacccgagtgcgcgctgagcgcccgctcgcggtcccgcggagcctccgcgttagtccccgccccgcgccgcgcagtcccccgggaggcatcgcgcacctctcgccgccccctcgcgcctcgccgattccccgcctccccttttccgcttcttcgccgcctccgctcgcggccgcgtcgcccgcgccccgctccctatctgctccccaggggggcactccgcaccttttgcgcccgctgccgccgccgcggccgccccgccgccctggtttcccccgcgagcgcggccgcgtcgccgcgcaaagactcgccgcgtgccgccccgagcaacgggtggcggcggcgcggcggcgggcggggcgcggcggcgcgtaggcggggctaggcgccggctaggcgaaacgccgcccccgggcgccgccgccgcccgctccagagcagtcgccgcgccagaccgccaacgcagagaccgagaccgaggtacgtcgcgcccgagcacgccgcgacgcgcggcagggacgaggagcacgacgccgcgccgcgccgcgcggggggggggagggagaggcaggacgcgggagcgagcgtgcatgtttccgcgcgagacgacgccgcgcgcgctggagaggagataaggcgcttggatcgcgagagggccagccaggctggaggcgaaaatgggtggagaggatagtatcttgcgtgcttggacgaggagactgacgaggaggacggatacgtcgatgatgatgtgcacagagaagaagcagttcgaaagcgactactagcaagcaagggatccatgaagttcgcgacctcggtcgcaattttgcttgtggccaacatagccaccgccctcgcgtcgatgaccaacgagacctcggaccgccctctcgtgcactttacccccaacaagggttggatgaacgatcccaacggcctctggtacgacgagaaggatgctaagtggcacctttactttcagtacaaccctaacgacaccgtctggggcaccccgctcttctggggccacgccacctccgacgacctcaccaactgggaggaccagcccattgctatcgcccccaagcgcaacgactcgggagctttttccggttccatggttgtggactacaacaacacctccggtttttttaacgacaccattgacccccgccagcgctgcgtcgccatctggacctacaacacgcccgagagcgaggagcagtacatcagctacagccttgatggaggctacacctttaccgagtaccagaagaaccctgtcctcgccgccaactccacccagttccgcgaccctaaggttttttggtacgagccttcccagaagtggattatgaccgccgctaagtcgcaggattacaagatcgagatctacagcagcgacgacctcaagtcctggaagcttgagtccgcctttgccaacgagggttttctcggataccagtacgagtgccccggtctcatcgaggtccccaccgagcaggacccgtccaagtcctactgggtcatgtttatttccatcaaccctggcgcccctgccggcggcagcttcaaccagtacttcgtcggctcctttaacggcacgcattttgaggccttcgacaaccagtcccgcgtcgtcgacttcggcaaggactactacgccctccagaccttctttaacaccgaccccacctacggcagcgccctcggtattgcttgggcctccaactgggagtactccgctttcgtccccactaacccctggcgcagctcgatgtccctcgtccgcaagttttcgcttaacaccgagtaccaggccaaccccgagaccgagcttattaacctgaaggccgagcctattctcaacatctccaacgctggcccctggtcccgctttgctactaacactaccctcaccaaggccaactcctacaacgtcgatctctccaactccaccggtactcttgagtttgagctcgtctacgccgtcaacaccacccagaccatctccaagtccgtcttcgccgacctctccctctggttcaagggccttgaggaccccgaggagtacctgcgcatgggttttgaggtctccgcctcctccttcttcctcgatcgcggtaactccaaggttaagtttgtcaaggagaacccctactttactaaccgtatgagcgtcaacaaccagccctttaagtccgagaacgatcttagctactacaaggtttacggcctcctcgaccagaacattctcgagctctactttaacgacggagatgtcgtcagcaccaacacctactttatgaccactggaaacgccctcggcagcgtgaacatgaccaccggagtcgacaacctcttttacattgacaagtttcaggttcgcgaggttaagtaacatatgttatgagagatccgaaagtgaaccttgtcctaacccgacagcgaatggcgggagggggcgggctaaaagatcgtattacatagtatttttcccctactctttgtgtttgtcttttttttttttttgaacgcattcaagccacttgtctgggtttacttgtttgtttgcttgcttgcttgcttgcttgcctgcttcttggtcagacggcccaaaaaagggaaaaaattcattcatggcacagataagaaaaagaaaaagtttgtcgaccaccgtcatcagaaagcaagagaagagaaacactcgcgctcacattctcgctcgcgtaagaatcttagccacgcatacgaagtaatttgtccatctggcgaatctttacatgagcgttttcaagctggagcgtgagatcatacctttcttgatcgtaatgttccaaccttgcataggcctcgttgcgatccgctagcaatgcgtcgtactcccgttgcaactgcgccatcgcctcattgtgacgtgagttcagattcttctcgagaccttcgagcgctgctaatttcgcctgacgctccttcttttgtgcttccatgacacgccgcttcaccgtgcgttccacttcttcctcagacatgcccttggctgcctcgacctgctcggtaagcttcgtcgtaatctcctcgatctcggaattcttcttgccctccatccactcggcaccatacttggcagcctgttcaacacgctcattgaaaaacttttcattctcttccagctccgcaacccgcgctcgaagctcattcacttccgccaccacggcttcggcatcgagcgccgaatcagtcgccgaactttccgaaagatacaccacggcccctccgctgctgctgcgcagcgtcatcatcagtcgcgtgttatcttcgcgcagattctccacctgctccgtaagcagcttcacggtggcctcttgattctgagggctcacgtcgtggattagcgcttgcagctcttgcagctccgtcagcttggaagagctcgtaatcatggctttgcacttgtccagacgtcgcagagcgttcgagagccgcttcgcgttatctgccatggacgcttctgcgctcgcggcctccctgacgacagtctcttgcagtttcactagatcatgtccaatcagcttgcggtgcagctctccaatcacgttctgcatcttgtttgtgtgtccgggccgcgcctcgtcttgcgatttgcgaatttcctcctcgagctcgcgttcgagctccagggcgcctttaagtagctcgaagtcagccgccgttagccccagctccgtcgccgcgttcagacagtcggttagcttgattcgattccgcttttccatggcaagtttaagatcctggcccagctgcacctcctgcgccttgcgcatcatgcgcggttccgcctggcgcaaaagcttcgagtcgtatcctgcctgccatgccagcgcaatggcacgcacgagcgacttgagttgccaactattcatcgccgagatgagcagcattttgatctgcatgaacacctcgtcagagtcgtcatcctctgcctcctccagctctgcgggcgagcgacgctctccttgcagatgaagcgagggccgcaggcctccgaagagcacctcttgcgcgagatcctcctccgtcgtcgccctccgcaggattgcggtcgtgtccgccatcttgccgccacagcagcttttgctcgctctgcaccttcaatttctggtgccgctggtgccgctggtgccgcttgtgctggtgctggtgctggtgctggtgctggtgccttgtgctggtgctgccacagacaccgccgctcctgctgctgctcttccggccccctcgccgccgccgcgagcccccgccgcgcgccgtgcctgggctctccgcgctctccgcgggctcctcggcctcggcctcgccgtccgcgacgacgtctgcgcggccgatggtgcggatctgctctagagggcccttcgaaggtaagcctatccctaaccctctcctcggtctcgattctacgcgtaccggtcatcatcaccatcaccattgagtttaaacgggccccagcacgtgctacgagatttcgattccaccgccgccttctatgaaaggttgggcttcggaatcgttttccgggacgccggctggatgatcctccagcgcggggatctcatgctggagttcttcgcccaccccaacttgtttattgcagcttataatggttacaaataaagcaatagcatcacaaatttcacaaataaagcatttttttcactgcattctagttgtggtttgtccaaactcatcaatgtatcttatcatacatggtcgacctgcaggaacctgcattaatgaatcggccaacgcgcggggagaggcggtttgcgtattgggcgctcttccgcttcctcgctcactgactcgctgcgctcggtcgttcggctgcggcgagcggtatcagctcactcaaaggcggtaatacggttatccacagaatcaggggataacgcaggaaagaacatgtgagcaaaaggccagcaaaaggccaggaaccgtaaaaaggccgcgttgctggcgtttttccataggctccgcccccctgacgagcatcacaaaaatcgacgctcaagtcagaggtggcgaaacccgacaggactataaagataccaggcgtttccccctggaagctccctcgtgcgctctcctgttccgaccctgccgcttaccggatacctgtccgcctttctcccttcgggaagcgtggcgctttctcatagctcacgctgtaggtatctcagttcggtgtaggtcgttcgctccaagctgggctgtgtgcacgaaccccccgttcagcccgaccgctgcgccttatccggtaactatcgtcttgagtccaacccggtaagacacgacttatcgccactggcagcagccactggtaacaggattagcagagcgaggtatgtaggcggtgctacagagttcttgaagtggtggcctaactacggctacactagaagaacagtatttggtatctgcgctctgctgaagccagttaccttcggaaaaagagttggtagctcttgatccggcaaacaaaccaccgctggtagcggtggtttttttgtttgcaagcagcagattacgcgcagaaaaaaaggatctcaagaagatcctttgatcttttctacggggtctgacgctcagtggaacgaaaactcacgttaagggattttggtcatgagattatcaaaaaggatcttcacctagatccttttaaattaaaaatgaagttttaaatcaatctaaagtatatatgagtaaacttggtctgacagttaccaatgcttaatcagtgaggcacctatctcagcgatctgtctatttcgttcatccatagttgcctgactccccgtcgtgtagataactacgatacgggagggcttaccatctggccccagtgctgcaatgataccgcgagacccacgctcaccggctccagatttatcagcaataaaccagccagccggaagggccgagcgcagaagtggtcctgcaactttatccgcctccatccagtctattaattgttgccgggaagctagagtaagtagttcgccagttaatagtttgcgcaacgttgttgccattgctacaggcatcgtggtgtcacgctcgtcgtttggtatggcttcattcagctccggttcccaacgatcaaggcgagttacatgatcccccatgttgtgcaaaaaagcggttagctccttcggtcctccgatcgttgtcagaagtaagttggccgcagtgttatcactcatggttatggcagcactgcataattctcttactgtcatgccatccgtaagatgcttttctgtgactggtgagtactcaaccaagtcattctgagaatagtgtatgcggcgaccgagttgctcttgcccggcgtcaatacgggataataccgcgccacatagcagaactttaaaagtgctcatcattggaaaacgttcttcggggcgaaaactctcaaggatcttaccgctgttgagatccagttcgatgtaacccactcgtgcacccaactgatcttcagcatcttttactttcaccagcgtttctgggtgagcaaaaacaggaaggcaaaatgccgcaaaaaagggaataagggcgacacggaaatgttgaatactcatactcttcctttttcaatattattgaagcatttatcagggttattgtctcatgagcggatacatatttgaatgtatttagaaaaataaacaaataggggttccgcgcacatttccccgaaaagtgccacctgacgtctaagaaaccattattatcatgacattaacctataaaaataggcgtatcacgaggccctttcgtctcgcgcgtttcggtgatgacggtgaaaacctctgacacatgcagctcccggagacggtcacagcttgtctgtaagcggatgccgggagcagacaagcccgtcagggcgcgtcagcgggtgttggcgggtgtcggggctggcttaactatgcggcatcagagcagattgtactgagagtgcaccaagctttgcctcaacgcaactaggcccaggcctactttcactgtgtcttgtcttgcctttcacaccgaccgagtgtgcacaaccgtgttttgcacaaagcgcaagatgctcactcgactgtgaagcaaaggttgcgcgcaagcgactgcgactgcgaggatgaggatgactggcagcctgttcaaaaactgaaaatccgcgatgggtcagctgccattcgcgcatgacgcctgcgagagacaagttaactcgtgtcactggcatgtcctagcatctttacgcgagcaaaattcaatcgctttattttttcagtttcgtaaccttctcgcaaccgcgaatcgccgtttcagcctgactaatctgcagctgcgtggcactgtcagtcagtcagtcagtcgtgcgcgctgttccagcaccgaggtcgcgcgtcgccgcgcctggaccgctgctgctactgctagtggcacggcaggtaggagcttgttgccggaacaccagcagccgccagtcgacgccagccaggggaaagtccggcgtcgaagggagaggaaggcggcgtgtgcaaactaacgttgaccactggcgcccgccgacacgagcaggaagcaggcagctgcagagcgcagcgcgcaagtgcagaatgcgcgaaagatccacttgcgcgcggcgggcgcgcacttgcgggcgcggcgcggaacagtgcggaaaggagcggtgcagacggcgcgcagtgacagtgggcgcaaagccgcgcagtaagcagcggcggggaacggtatacgcagtgccgcgggccgccgcacacagaagtatacgcgggccgaagtggggcgtcgcgcgcgggaagtgcggaatggcgggcaaggaaaggaggagacggaaagagggcgggaaagagagagagagagagtgaaaaaagaaagaaagaaagaaagaaagaaagaaagctcggagccacgccgcggggagagagagaaatgaaagcacggcacggcaaagcaaagcaaagcagacccagccagacccagccgagggaggagcgcgcgcaggacccgcgcggcgagcgagcgagcacggcgcgcgagcgagcgagcgagcgagcgcgcgagcgagcaaggcttgctgcgagcgatcgagcgagcgagcgggaaggatgagcgcgacccgcgcggcgacgaggacagcggcggcgctgtcctcggcgctgacgacgcctgtaaagcagcagcagcagcagcagctgcgcgtaggcgcggcgtcggcacggctggcggccgcggcgttctcgtccggcacgggcggagacgcggccaagaaggcggccgcggcgagggcgttctccacgggacgcggccccaacgcgacacgcgagaagagctcgctggccacggtccaggcggcgacggacgatgcgcgcttcgtcggcctgaccggcgcccaaatctttcatgagctcatgcgcgagcaccaggtggacaccatctttggctaccctggcggcgccattctgcccgtttttgatgccatttttgagagtgacgcgcttcaagttcattctcgctcgccacgagcagggcgccggccacatggccgagggctacgcgcgcgccacgggcaagcccggcgttgtcctcgtcacctcgggccctggagccaccaacaccatcaccccgatcatggatgcttacatggacggtacgccgctgctcgtgttcaccggccaggtgcagacctctgctgtcggcacggacgctttccaggagtgtgacattgttggcatcagccgcgcgtgcaccaagtggaacgtcatggtcaaggacgtgaaggagctcccgcgccgcatcaatgaggcctttgagattgccatgagcggccgcccgggtcccgtgctcgtcgatcttcctaaggatgtgaccgccgttgagctcaaggaaatgcccgacagctccccccaggttgctgtgcgccagaagcaaaaggtcgagcttttccacaaggagcgcattggcgctcctggcacggccgacttcaagctcattgccgagatgatcaaccgtgcggagcgacccgtcatctatgctggccagggtgtcatgcagagcccgttgaatggcccggctgtgctcaaggagttcgcggagaaggccaacattcccgtgaccaccaccatgcagggtctcggcggctttgacgagcgtagtcccctctccctcaagatgctcggcatgcacggctctgcctacgccaactactcgatgcagaacgccgatcttatcctggcgctcggtgcccgctttgatgatcgtgtgacgggccgcgttgacgcctttgctccggaggctcgccgtgccgagcgcgagggccgcggtggcatcgttcactttgagatttcccccaagaacctccacaaggtcgtccagcccaccgtcgcggtcctcggcgacgtggtcgagaacctcgccaacgtcacgccccacgtgcagcgccaggagcgcgagccgtggtttgcgcagatcgccgattggaaggagaagcacccttttctgctcgagtctgttgattcggacgacaaggttctcaagccgcagcaggtcctcacggagcttaacaagcagattctcgagattcaggagaaggacgccgaccaggaggtctacatcaccacgggcgtcggaagccaccagatgcaggcagcgcagttccttacctggaccaagccgcgccagtggatctcctcgggtggcgccggcactatgggctacggccttccctcggccattggcgccaagattgccaagcccgatgctattgttattgacatcgatggtgatgcttcttattcgatgaccggtatggaattgatcacagcagccgaattcaaggttggcgtgaagattcttcttttgcagaacaactttcagggcatggtcaagaacgttcaggatctcttttacgacaagcgctactcgggccaccgccatgttcaacccgcgcttcgacaaggtcgccgatgcgatgcgtgccaagggtctctactgcgcgaaacagtcggagctcaaggacaagatcaaggagtttctcgagtacgatgagggtcccgtcctcctcgaggttttcgtggacaaggacacgctcgtcttgcccatggtccccgctggctttccgctccacgagatggtcctcgagcctcctaagcccaaggacgcctaagttcttttttccatggcgggcgagcgagcgagcgcgcgagcgcgcaagtgcgcaagcgccttgccttgctttgcttcgcttcgctttgctttgcttcacacaacctaagtatgaattcaagttttcttgcttgtcggcgatgcctgcctgccaaccagccagccatccggccggccgtccttgacgccttcgcttccggcgcggccatcgattcaattcacccatccgatacgttccgccccctcacgtccgtctgcgcacgacccctgcacgaccacgccaaggccaacgcgccgctcagctcagcttgtcgacgagtcgcacgtcacatatctcagatgcatttggactgtgagtgttattatgccactagcacgcaacgatcttcggggtcctcgctcattgcatccgttcgggccctgcaggcgtggacgcgagtcgccgccgagacgctgcagcaggccgctccgacgcgagggctcgagctcgccgcgcccgcgcgatgtctgcctggcgccgactgatctctggagcgcaaggaagacacggcgacgcgaggaggaccgaagagagacgctggggtatgcaggatatacccggggcgggacattcgttccgcatacactcccccattcgagcttgctcgtccttggcagagccgagcgcgaacggttccgaacgcggcaaggattttggctctggtgggtggactccgatcgaggcgcaggttctccgcaggttctcgcaggccggcagtggtcgttagaaatagggagtgccggagtcttgacgcgccttagctcactctccgcccacgcgcgcatcgccgccatgccgccgtcccgtctgtcgctgcgctggccgcgaccggctgcgccagagtacgacagtgggacagagctcgaggcgacgcgaatcgctcgggttgtaagggtttcaagggtcgggcgtcgtcgcgtgccaaagtgaaaatagtaggggggggggggggtac

SEQ ID NO: 59 - protein, 32 aa, Schizochytrium
MRTVRGPQTAALAALLALAATHVAVSPFTKVE

SEQ ID NO: 60 - DNA, 96 bp, Schizochytrium
atgcgcacggtgagggggccgcaaacggcggcactcgccgcccttctggcacttgccgcgacgcacgtggctgtgagcccgttcaccaaggtggag

SEQ ID NO: 61 - protein, 30 aa, Schizochytrium
MGRLAKSLVLLTAVLAVIGGVRAEEDKSEA

SEQ ID NO: 62 - DNA, 90 bp, Schizochytrium
atgggccgcctcgcgaagtcgcttgtgctgctgacggccgtgctggccgtgatcggaggcgtccgcgccgaagaggacaagtccgaggcc

SEQ ID NO: 63 - protein, 38 aa, Schizochytrium
MTSTARALALVRALVLALAVLALLASQSVAVDRKKFRT

SEQ ID NO: 64 - DNA, 114 bp, Schizochytrium
atgacgtcaacggcgcgcgcgctcgcgctcgtgcgtgctttggtgctcgctctggctgtcttggcgctgctagcgagccaaagcgtggccgtggaccgcaaaaagttcaggacc

SEQ ID NO: 65 - protein, 34 aa, Schizochytrium
MLRLKPLLLLFLCSLIASPVVAWARGGEGPSTSE

SEQ ID NO: 66 - DNA, 102 bp, Schizochytrium
atgttgcggctcaagccacttttactcctcttcctctgctcgttgattgcttcgcctgtggttgcctgggcaagaggaggagaagggccgtccacgagcgaa

SEQ ID NO: 67 - protein, 29 aa, Schizochytrium
MAKILRSLLLAAVLVVTPQSLRAHSTRDA

SEQ ID NO: 68 - DNA, 87 bp, Schizochytrium
atggccaagatcttgcgcagtttgctcctggcggccgtgctcgtggtgactcctcaatcactgcgtgctcattcgacgcgggacgca

SEQ ID NO: 69 - protein, 36 aa, Schizochytrium
MVFRRVPWHGAATLAALVVACATCLGLGLDSEEATY

SEQ ID NO: 70 - DNA, 108 bp, Schizochytrium
atggtgtttcggcgcgtgccatggcacggcgcggcgacgctggcggccttggtcgtggcctgcgcgacgtgtttaggcctgggactggactcggaggaggccacgtac

SEQ ID NO: 71 - protein, 30 aa, Schizochytrium
MTANSVKISIVAVLVAALAWETCAKANYQW

SEQ ID NO: 72 - DNA, 90 bp, Schizochytrium
atgacagctaactcggtgaaaataagcatcgtggctgtgctggtcgcggcactggcttgggaaacatgcgcaaaagctaactatcagtgg

SEQ ID NO: 73 - protein, 35 aa, Schizochytrium
MARRASRLGAAVVVVLVVVASACCWQAAADVVDAQ

SEQ ID NO: 74 - DNA, 105 bp, Schizochytrium
atggcgcgcagggcgtcgcgcctcggcgccgccgtcgtcgtcgtcctcgtcgtcgtcgcctccgcctgctgctggcaagccgctgcggacgtcgtggacgcgcag

SEQ ID NO: 75 - DNA, 1785 bp, Artificial Sequence
  Codon optimized nucleic acid sequence
atgaagttcgcgacctcggtcgcaattttgcttgtggccaacatagccaccgccctcgcggcctccccctcgatgcagacccgtgcctccgtcgtcattgattacaacgtcgctcctcctaacctctccaccctcccgaacggcagcctctttgagacctggcgtcctcgcgcccacgttcttccccctaacggtcagattggcgatccctgcctccactacaccgatccctcgactggcctctttcacgtcggctttctccacgatggctccggcatttcctccgccactactgacgacctcgctacctacaaggatctcaaccagggcaaccaggtcatcgtccccggcggtatcaacgaccctgtcgctgttttcgacggctccgtcattccttccggcattaacggcctccctaccctcctctacacctccgtcagctacctccccattcactggtccatcccctacacccgcggttccgagacgcagagcctggctgtctccagcgatggtggctccaactttactaagctcgaccagggccccgttattcctggccccccctttgcctacaacgtcaccgccttccgcgacccctacgtctttcagaaccccaccctcgactccctcctccactccaagaacaacacctggtacaccgtcatttcgggtggcctccacggcaagggccccgcccagtttctttaccgtcagtacgaccccgactttcagtactgggagttcctcggccagtggtggcacgagcctaccaactccacctggggcaacggcacctgggccggccgctgggccttcaacttcgagaccggcaacgtcttttcgcttgacgagtacggctacaacccccacggccagatcttctccaccattggcaccgagggctccgaccagcccgttgtcccccagctcacctccatccacgatatgctttgggtctccggtaacgtttcgcgcaacggatcggtttccttcactcccaacatggccggcttcctcgactggggtttctcgtcctacgccgccgcgggtaaggttcttccttccacgtcgctcccctccaccaagtccggtgcccccgatcgcttcatttcgtacgtttggctctccggcgacctctttgagcaggctgagggctttcctaccaaccagcagaactggaccggcaccctcctcctcccccgtgagctccgcgtcctttacatccccaacgtggttgataacgcccttgcgcgcgagtccggcgcttcctggcaggtcgtctcctccgatagctcggccggtactgtggagctccagaccctcggcatttccatcgcccgcgagaccaaggccgccctcctgtccggcacctcgttcactgagtccgaccgcactcttaactcctccggcgtcgttccctttaagcgttccccctccgagaagtttttcgtcctctccgcccagctctccttccccgcctccgcccgcggctcgggcctcaagtccggcttccagattctttcctccgagctcgagtccaccacggtctactaccagtttagcaacgagtccatcatcgtcgaccgcagcaacaccagcgccgccgcccgtactaccgacggtatcgactcctccgccgaggccggcaagctccgcctctttgacgtcctcaacggcggcgagcaggctattgagaccctcgaccttaccctcgtcgttgataactccgtgctcgagatttacgccaacggtcgtttcgcgctttccacctgggttcgctaa

SEQ ID NO: 76 - DNA, 1682 bp, Artificial Sequence
  Codon Optimized HA
atgaaggctaacctcctcgttcttctttccgctctcgctgctgcggatgccgacaccatctgcattggctaccacgctaacaacagcacggacaccgtcgatactgtcctggagaagaacgttaccgcacccattcggtcaacctcctggaggacagccacaacggcaagctctgccgtcttaagggcatcgcccccctccagctcggcaagtgcaacatcgccggctggctcctcggcaacccggagtgcgatccctcctccccgttcgctcctggtcgtacattgtggagactccgaacagcgagaacggtatctgctaccccggcgattttatcgactacgaggagctccgcgagcagctctcctccgtgtccagcttgagcgtttcgagatttttccgaaggagtcctcgtggcccaaccacaacaccaacggcgtcaccgccgcctgctcccacgagggcaagtcgagcttttaccgcaacctgctttggctcaccgagaagggggttcgtaccctaagctcaagaactcgtacgtcaacaagaagggcaaggaggtcctcgtcctctggggcatccaccatcccccgaacagcaaggagcagcagaacatctaccagaacgagaacgccacgtttcggtggtcacgtcgaactacaaccgccgcttcactcctgagatcgccgagcgccccaaggtgcgcgaccaggctggccgcatgaactactactggaccctccttaagcccggtgacacgatatctttgaggccaacggcaaccttatcgcgcccatgtacgcgttcgccctctcccgcggctttggtagcggcatcattaccagcaacgccagcatgcacgagtgcaacacgaagtgccagaccccgccggtgccatcaacagcagcctgccttaccagaacatccaccccgtcaccatcggtgagtgcccgaagtacgtgcgctcggccaagctccgcatggtcacgggcctccgcaacactccttcgatccagcccgcggcctcttcggcgccattgccggtttcatcgagggcggctggacgggcatgatcgacggctggtacggctaccaccaccagaacgagcagggctccggttacgccgcggaccagaagtccaccagaacgccatcaacggcattactaacaaggtcaacacggtcatcgagaagatgaacattcagtttaccgctgtcggcaaggagttcaacaagctggagaagcgcatggagaacctcaacaagaaggggacgatggtttcctggacatttggacctacaacgccgagctcctcgtgctccttgagaacgagcgtaccctcgacttccacgactccaacgtcaagaacctctacgagaaggtcaagtcgcagctcagaacaacgccaaggagattggcaacggttgcttcgagttttaccacaagtgcgacaacgagtgcatggagtccgtccgcaacggcacctacgactacccgaagtactccgaggagtcgaagctgaacgcgagaaggtggacggcgtgaagctggagtccatgggcatctaccagatcctcgccatttactcgacggttgcctcgtcgctcgtcctccttgtctccctcggtgcgatttcgttctggatgtgctgaacggcagccttcagtgccgcatctgcatc

SEQ ID NO: 77 - protein, 565 aa, Influenza A virus
MKANLLVLLSALAAADADTICIGYHANNSTDTVDTVLEKNVTVTHSVNLLEDSHNGKLCRLKGIAPLQLGKCNIAGWLLGNPECDPLLPVRSWSYIVETPNSENGICYPGDFIDYEELREQLSSVSSFERFEIFPKESSWPNHNTNGVTAACSHEGKSSFYRNLLWLTEKEGSYPKLKNSYVNKKGKEVLVLWGIHHPPNSKEQQNIYQNENAYVSVVTSNYNRRFTPEIAERPKVRDQAGRMNYYWTLLKPGDTIIFEANGNLIAPMYAFALSRGFGSGIITSNASMHECNTKCQTPLGAINSSLPYQNIHPVTIGECPKYVRSAKLRMVTGLRNTPSIQSRGLFGAIAGFIEGGWTGMIDGWYGYHHQNEQGSGYAADQKSTQNAINGITNKVNTVIEKMNIQFTAVGKEFNKLEKRMENLNKKVDDGFLDIWTYNAELLVLLENERTLDFHDSNVKNLYEKVKSQLKNNAKEIGNGCFEFYHKCDNECMESVRNGTYDYPKYSEESKLNREKVDGVKLESMGIYQILAIYSTVASSLVLLVSLGAISFWMCSNGSLQCRICI

SEQ ID NO: 78 - protein, 51 aa, Schizochytrium
  GlcNac-transferase-I-like protein
MRGPGMVGLSRVDREHLRRRQQQAASEWRRWGFFVATAVVLLVFLTVYPNV

SEQ ID NO: 79 - DNA, 153 bp, Schizochytrium
  signal anchor sequence
atgcgcggcccgggcatggtcggcctcagccgcgtggaccgcgagcacctgcggcggcggcagcagcaggcggcgagcgaatggcggcgctgggggttcttcgtcgcgacggccgtcgtcctgctcgtctttctcaccgtatacccgaacgta

SEQ ID NO: 80 - protein, 66 aa, Schizochytrium
  beta-1,2- xylosyltransferase-like protein
MRTRGAAYVRPGQHEAKALSSRSSDEGYTTVNVVRTKRKRTTVAALVAAALLVTGFIVVVVFVVVV

SEQ ID NO: 81 - DNA, 198 bp, Schizochytrium
  signal anchor sequence
atgcgcacgcggggcgcggcgtacgtgcggccgggacagcacgaggcgaaggcgctctcgtcaaggagcagcgacgagggatatacgacggtcaacgttgtcaggaccaagcgaaagaggaccactgtagccgcgcttgtagccgcggcgctgctggtgacgggctttatcgtcgtcgtcgtcttcgtcgtcgttgtt

SEQ ID NO: 82 - protein, 64 aa, Schizochytrium
  beta-1,4-xylosidase-like protein
MEALREPLAAPPTSARSSVPAPLAKEEGEEEDGEKGTFGAGVLGVVAVLVIVVFAIVAGGGGDI

SEQ ID NO: 83 - DNA, 192 bp, Schizochytrium
  signal anchor sequence
atggaggccctgcgcgagcccttggctgcgccgccaacgtcggcgcgatcgtcggtgccagcgccgctcgcgaaggaggagggggaggaggaggacggggaaaaagggacgtttggggcgggggtcctcggtgtcgtggcggtgctcgtcatcgtggtgtttgcgatcgtggcgggaggcggaggcgatatt

SEQ ID NO: 84 - protein, 73 aa, Schizochytrium
  galactosyltransferase-like protein
MLSVAQVAGSAHSRPRRGGERMQDVLALEESSRDRKRATARPGLYRALAILGLPLIVFIVWQMTSSLTTAPSA

SEQ ID NO: 85 - DNA, 219 bp, Schizochytrium
  signal anchor sequence
atgttgagcgtagcacaagtcgcggggtcggcccactcgcggccgagacgaggtggtgagcggatgcaagacgtgctggccctggaggaaagcagcagagatcgaaaacgagcaacagcaaggcccgggctatatcgcgcacttgcgattctggggctgccgctcatcgtattcatcgtatggcaaatgactagctccctcacgactgccccgagcgcc

SEQ ID NO: 86 - protein, 997 aa, Schizochytrium
  EMC1
MGTTTARMAVAVLAAAVSVAHGLHEDQAGVNDWTVRNLGAYAHGVFLDDDLALVATTQATVGAVRMTDGEVVWRETLPTARSAPLASQVKHELFATASADACVIELWATPSGDVMTSDSRQAGLEWDAKICDNTDADATGVLELLDNDFNNDGTPDVAALTPFQFVILDGVSGRVLHEVDLDKTIAWQGLVEAAGSATGGKRKRPSIMAYGVDIKTGKLEVRKLANSGATLDPVSGLEGVSADEITVLKSGVAKVGSALLFVRKESGALVAFDCVANQLQELTNAPSIKGSVQSLGSARFFATDAGVIYAVDGELKIAETLKGVEAAAIGVSGASVIAAVQSSTASGTGDEAQCGPISRVLVQSASGVTEIAFPEQQGQSGARGLVEKIIVGDSSTGTRAIFVFEDASAVGIEIESGASEASTLFVREEALANVVEAVAVDLPPTDEVGSLGDEAAHVFAHGSHASIFMFRLKDQVRTVQRFVQSLFGAATQHLSEFVASQGKTLVQAIRGELPRAESLSQSEMFSFGFRRVLVLRSASGKVFGLNSADGSLLWAAQSPGSRLFVTRAREAGLDHPAEVAIVDEAHGRVTWRNAITGAVTRVEDIDTPLAQIAVLPGDIFPSTASSEEDVSPAAVLIALDHAQRVHILPSSRTESVLQLEDLLRALHFVVYSNETGALTGYAVDPSQRAGVELWSMIVPASQTLLAVEGQSGGALNNPGIKRGDGAVLVKFVDPHLLMVATQSGPHLQVSILNGISGRVISRFTHKKSTGPVHAVLADNTVTYSFWNQVKSRQEVSVVGLFEGEIGPRELNMWSSRPNMGSGKAMSAFDDSMMPNVQQKTFYTERAIAALGVTKTRFGIADRRVLIGTANGAVNMQVPQILSPRRPVGKLSDMEKEEGLMLYAPELPLIPTQTITYYESIPQLRLIRSFATRLESTSLVLAAGLDIFYTRVMPSRGFDVLDEDFASGLLLALIAALLALTIYLSKAVGKSTLDETWK

SEQ ID NO: 87 - protein, 731 aa, Schizochytrium
  Nicastrin-like
MGAARRSMGAARKALAASATLAALALAGLQPARAEVNGVNAMTEAMLTEYASLPCVRSIARDGAVGCGSPSDRSVAEGGALFLVESVEDVTGLIENAQGLDAVALVVDDALLHGDSLRAMQDLAKKIRVTAVIVTVEEDGSPQEPPRSSAAPTTWIPSGDGLLNETVSFVVTRLRNATQSEEIRALAASNRDRGYVDAVFQHSARYQFYLGKETATSLSCLASGRCDPLGGLSVWASAGPVPVNSAKETVLLTANLDAASFFHDVVPARDTTASGVAAVLLAAKALASVDESVLEALSKQIAVALFNGEVWSRAGSRRFVHDVALGECLSPQTASPYNESTCANPPVYALAWTSLGLDNITDVVSVNNVAGSESGAFYVHTAAGTASANAAAALQSVASSSTDVDVSITGATTSGVVPPSPLDSFLAAEMETDVSFSGAGLVVSGFDAAITDANPRYSSRYDRRDKGPEADDAEALTAARIADVATLLARHAFVQAGGSISDAVNFVLVDGTHAAELWDCLTKDFACTLVADVIGAEDTTAVADFMGSTLLAASEGVAGGAPNFFSGIYSPFPVENNVMRPVPLFVRDYLAQYGRNASLIEKVTESAKYACAQDLDCMVMTEPPACELGRSALACLRGGCVCSNAYFHDAVSPALVYEDGAFSVDAQKLTDDDGLWTEPRWSDGTLTLYTSANSASTTIALLVCGILLTIGCVFALRKAQGMLDNTKYKLN

SEQ ID NO: 88 - protein, 232 aa, Schizochytrium
  Emp24
MATTENEARLPPGKQRLGRRRRGRVSKASGWGTTLALAAAVLVFSVDRASGVRFEVASTEERCIFDVLRKDQLVTGEFEVHADGDDVNMDIHVTGPLGEEVFSKQNSKMAKFGFTAEAAGEHVLCLRNNDMIMREVQVKLRSGVEAKDLTEVVQRHHLKPLSAEVIRIQETIRDVRHELTALKQREAEMRDMNESINTRVSLFSFFSIAVVGSLGAWQIMYLKSYFQRKKLI

SEQ ID NO: 89 - protein, 550 aa, Schizochytrium
  Calnexin-like
MRTTFVAAYAAVAALALGQCEAINFRESFEGANVEKEWVKSASDRYAGSEWAFDTSKDTGDVGLQTVKPHKFYGISRKFENPIPVGDGEKPFVAQYEVKFTEGVSCSGAYLKLLEQDDAFTPKDLVESSPYSIMFGPDNCGANNKVHLIFRQENPVTKEYEEKHMTKKVTSVRDRTSHVYTLEVHPDNTFKVKVDGKVEAEGSLTDDEAFSPPFQQPKEIDDPNDEKPDDWVDQAKIPDPEASKPDDWDEDAPKRIADPDAVKPEGWLDDEPDQVPDPAASEPEDWDEEDDGIWEAPLVANPKCTAGPGCGEWNAPMIENPNYKGKWSAPMIDNPEYKGVWKPRRIENPAYFEESSPVTTIKPIGAVAIEILANDKGIRFDNIIIGNDVKEAAEFIDKEFLAKQADEKAKVKEEAAQAAQNSRWEEYKKGSIQGYVMWYAGDYIDYVMELYEASPIAVGVGAAAAGLAVLVALMVMCMSGAPEEYDDDVALHKKDDDAAAGDDDEAEAEAENDAADEDEDEEDDDDEEDEDEEEDEDEATGPRRRVNRAN

SEQ ID NO: 90 - DNA, 6175 bp, Artificial
  pCL0121
ctcttatctgcctcgcgccgttgaccgccgcttgactcttggcgcttgccgctcgcatcctgcctcgctcgcgcaggcgggcgggcgagtgggtgggtccgcagccttccgcgctcgcccgctagctcgctcgcgccgtgctgcagccagcagggcagcaccgcacggcaggcaggtcccggcgcggatcgatcgatccatcgatccatcgatccatcgatcgtgcggtcaaaaagaaaggaagaagaaaggaaaaagaaaggcgtgcgcacccgagtgcgcgctgagcgcccgctcgcggtcccgcggagcctccgcgttagtccccgccccgcgccgcgcagtcccccgggaggcatcgcgcacctctcgccgccccctcgcgcctcgccgattccccgcctccccttttccgcttcttcgccgcctccgctcgcggccgcgtcgcccgcgccccgctccctatctgctccccaggggggcactccgcaccttttgcgcccgctgccgccgccgcggccgccccgccgccctggtttcccccgcgagcgcggccgcgtcgccgcgcaaagactcgccgcgtgccgccccgagcaacgggtggcggcggcgcggcggcgggcggggcgcggcggcgcgtaggcggggctaggcgccggctaggcgaaacgccgcccccgggcgccgccgccgcccgctccagagcagtcgccgcgccagaccgccaacgcagagaccgagaccgaggtacgtcgcgcccgagcacgccgcgacgcgcggcagggacgaggagcacgacgccgcgccgcgccgcgcggggggggggagggagaggcaggacgcgggagcgagcgtgcatgtttccgcgcgagacgacgccgcgcgcgctggagaggagataaggcgcttggatcgcgagagggccagccaggctggaggcgaaaatgggtggagaggatagtatcttgcgtgcttggacgaggagactgacgaggaggacggatacgtcgatgatgatgtgcacagagaagaagcagttcgaaagcgactactagcaagcaagggatccatgaagttcgcgacctcggtcgcaattttgcttgtggccaacatagccaccgccctcgcgcagagcgatggctgcacccccaccgaccagacgatggtgagcaagggcgaggagctgttcaccggggtggtgcccatcctggtcgagctggacggcgacgtaaacggccacaagttcagcgtgtccggcgagggcgagggcgatgccacctacggcaagctgaccctgaagttcatctgcaccaccggcaagctgcccgtgccctggcccaccctcgtgaccaccctgacctacggcgtgcagtgcttcagccgctaccccgaccacatgaagcagcacgacttcttcaagtccgccatgcccgaaggctacgtccaggagcgcaccatcttcttcaaggacgacggcaactacaagacccgcgccgaggtgaagttcgagggcgacaccctggtgaaccgcatcgagctgaagggcatcgacttcaaggaggacggcaacatcctgggacacaagctggagtacaactacaacagccacaacgtctatatcatggccgacaagcagaagaacggcatcaaggtgaacttcaagatccgccacaacatcgaggacggcagcgtgcagctcgccgaccactaccagcagaacacccccatcggcgacggccccgtgctgctgcccgacaaccactacctgagcacccagtccgccctgagcaaagaccccaacgagaagcgcgatcacatggtcctgctggagttcgtgaccgccgccgggatcactctcggcatggacgagctgtacaagcaccaccatcaccaccactaacatatgagttatgagatccgaaagtgaaccttgtcctaacccgacagcgaatggcgggagggggcgggctaaaagatcgtattacatagtatttttcccctactctttgtgtttgtcttttttttttttttgaacgcattcaagccacttgtctgggtttacttgtttgtttgcttgcttgcttgcttgcttgcctgcttcttggtcagacggcccaaaaaagggaaaaaattcattcatggcacagataagaaaaagaaaaagtttgtcgaccaccgtcatcagaaagcaagagaagagaaacactcgcgctcacattctcgctcgcgtaagaatcttagccacgcatacgaagtaatttgtccatctggcgaatctttacatgagcgttttcaagctggagcgtgagatcatacctttcttgatcgtaatgttccaaccttgcataggcctcgttgcgatccgctagcaatgcgtcgtactcccgttgcaactgcgccatcgcctcattgtgacgtgagttcagattcttctcgagaccttcgagcgctgctaatttcgcctgacgctccttcttttgtgcttccatgacacgccgcttcaccgtgcgttccacttcttcctcagacatgcccttggctgcctcgacctgctcggtaaaacgggccccagcacgtgctacgagatttcgattccaccgccgccttctatgaaaggttgggcttcggaatcgttttccgggacgccggctggatgatcctccagcgcggggatctcatgctggagttcttcgcccaccccaacttgtttattgcagcttataatggttacaaataaagcaatagcatcacaaatttcacaaataaagcatttttttcactgcattctagttgtggtttgtccaaactcatcaatgtatcttatcatacatggtcgacctgcaggaacctgcattaatgaatcggccaacgcgcggggagaggcggtttgcgtattgggcgctcttccgcttcctcgctcactgactcgctgcgctcggtcgttcggctgcggcgagcggtatcagctcactcaaaggcggtaatacggttatccacagaatcaggggataacgcaggaaagaacatgtgagcaaaaggccagcaaaaggccaggaaccgtaaaaaggccgcgttgctggcgtttttccataggctccgcccccctgacgagcatcacaaaaatcgacgctcaagtcagaggtggcgaaacccgacaggactataaagataccaggcgtttccccctggaagctccctcgtgcgctctcctgttccgaccctgccgcttaccggatacctgtccgcctttctcccttcgggaagcgtggcgctttctcatagctcacgctgtaggtatctcagttcggtgtaggtcgttcgctccaagctgggctgtgtgcacgaaccccccgttcagcccgaccgctgcgccttatccggtaactatcgtcttgagtccaacccggtaagacacgacttatcgccactggcagcagccactggtaacaggattagcagagcgaggtatgtaggcggtgctacagagttcttgaagtggtggcctaactacggctacactagaagaacagtatttggtatctgcgctctgctgaagccagttaccttcggaaaaagagttggtagctcttgatccggcaaacaaaccaccgctggtagcggtggtttttttgtttgcaagcagcagattacgcgcagaaaaaaaggatctcaagaagatcctttgatcttttctacggggtctgacgctcagtggaacgaaaactcacgttaagggattttggtcatgagattatcaaaaaggatcttcacctagatccttttaaattaaaaatgaagttttaaatcaatctaaagtatatatgagtaaacttggtctgacagttaccaatgcttaatcagtgaggcacctatctcagcgatctgtctatttcgttcatccatagttgcctgactccccgtcgtgtagataactacgatacgggagggcttaccatctggccccagtgctgcaatgataccgcgagacccacgctcaccggctccagatttatcagcaataaaccagccagccggaagggccgagcgcagaagtggtcctgcaactttatccgcctccatccagtctattaattgttgccgggaagctagagtaagtagttcgccagttaatagtttgcgcaacgttgttgccattgctacaggcatcgtggtgtcacgctcgtcgtttggtatggcttcattcagctccggttcccaacgatcaaggcgagttacatgatcccccatgttgtgcaaaaaagcggttagctccttcggtcctccgatcgttgtcagaagtaagttggccgcagtgttatcactcatggttatggcagcactgcataattctcttactgtcatgccatccgtaagatgcttttctgtgactggtgagtactcaaccaagtcattctgagaatagtgtatgcggcgaccgagttgctcttgcccggcgtcaatacgggataataccgcgccacatagcagaactttaaaagtgctcatcattggaaaacgttcttcggggcgaaaactctcaaggatcttaccgctgttgagatccagttcgatgtaacccactcgtgcacccaactgatcttcagcatcttttactttcaccagcgtttctgggtgagcaaaaacaggaaggcaaaatgccgcaaaaaagggaataagggcgacacggaaatgttgaatactcatactcttcctttttcaatattattgaagcatttatcagggttattgtctcatgagcggatacatatttgaatgtatttagaaaaataaacaaataggggttccgcgcacatttccccgaaaagtgccacctgacgtctaagaaaccattattatcatgacattaacctataaaaataggcgtatcacgaggccctttcgtctcgcgcgtttcggtgatgacggtgaaaacctctgacacatgcagctcccggagacggtcacagcttgtctgtaagcggatgccgggagcagacaagcccgtcagggcgcgtcagcgggtgttggcgggtgtcggggctggcttaactatgcggcatcagagcagattgtactgagagtgcaccaagcttccaattttaggccccccactgaccgaggtctgtcgataatccacttttccattgattttccaggtttcgttaactcatgccactgagcaaaacttcggtctttcctaacaaaagctctcctcacaaagcatggcgcggcaacggacgtgtcctcatactccactgccacacaaggtcgataaactaagctcctcacaaatagaggagaattccactgacaactgaaaacaatgtatgagagacgatcaccactggagcggcgcggcggttgggcgcggaggtcggcagcaaaaacaagcgactcgccgagcaaacccgaatcagccttcagacggtcgtgcctaacaacacgccgttctaccccgccttcttcgcgccccttcgcgtccaagcatccttcaagtttatctctctagttcaacttcaagaagaacaacaccaccaacaccatggccaagttgaccagtgccgttccggtgctcaccgcgcgcgacgtcgccggagcggtcgagttctggaccgaccggctcgggttctcccgggacttcgtggaggacgacttcgccggtgtggtccgggacgacgtgaccctgttcatcagcgcggtccaggaccaggtggtgccggacaacaccctggcctgggtgtgggtgcgcggcctggacgagctgtacgccgagtggtcggaggtcgtgtccacgaacttccgggacgcctccgggccggccatgaccgagatcggcgagcagccgtgggggcgggagttcgccctgcgcgacccggccggcaactgcgtgcacttcgtggccgaggagcaggactgacacgtgctacgagatttcgattccaccgccgccttctatgaaaggttgggcttcggaatcgttttccgggacgccggctggatgatcctccagcgcggggatctcatgctggagttcttcgcccaccccaacttgtttattgcagcttataatggttacaaataaagcaatagcatcacaaatttcacaaataaagcatttttttcactgcattctagttgtggtttgtccaaactcatcaatgtatcttatcggtac

SEQ ID NO: 91 - DNA, 6611 bp, Artificial
  pCL0122
ctcttatctgcctcgcgccgttgaccgccgcttgactcttggcgcttgccgctcgcatcctgcctcgctcgcgcaggcgggcgggcgagtgggtgggtccgcagccttccgcgctcgcccgctagctcgctcgcgccgtgctgcagccagcagggcagcaccgcacggcaggcaggtcccggcgcggatcgatcgatccatcgatccatcgatccatcgatcgtgcggtcaaaaagaaaggaagaagaaaggaaaaagaaaggcgtgcgcacccgagtgcgcgctgagcgcccgctcgcggtcccgcggagcctccgcgttagtccccgccccgcgccgcgcagtcccccgggaggcatcgcgcacctctcgccgccccctcgcgcctcgccgattccccgcctccccttttccgcttcttcgccgcctccgctcgcggccgcgtcgcccgcgccccgctccctatctgctccccaggggggcactccgcaccttttgcgcccgctgccgccgccgcggccgccccgccgccctggtttcccccgcgagcgcggccgcgtcgccgcgcaaagactcgccgcgtgccgccccgagcaacgggtggcggcggcgcggcggcgggcggggcgcggcggcgcgtaggcggggctaggcgccggctaggcgaaacgccgcccccgggcgccgccgccgcccgctccagagcagtcgccgcgccagaccgccaacgcagagaccgagaccgaggtacgtcgcgcccgagcacgccgcgacgcgcggcagggacgaggagcacgacgccgcgccgcgccgcgcggggggggggagggagaggcaggacgcgggagcgagcgtgcatgtttccgcgcgagacgacgccgcgcgcgctggagaggagataaggcgcttggatcgcgagagggccagccaggctggaggcgaaaatgggtggagaggatagtatcttgcgtgcttggacgaggagactgacgaggaggacggatacgtcgatgatgatgtgcacagagaagaagcagttcgaaagcgactactagcaagcaagggatccatgaagttcgcgacctcggtcgcaattttgcttgtggccaacatagccaccgccctcgcgcagagcgatggctgcacccccaccgaccagacgatggtgagcaagggcgaggagctgttcaccggggtggtgcccatcctggtcgagctggacggcgacgtaaacggccacaagttcagcgtgtccggcgagggcgagggcgatgccacctacggcaagctgaccctgaagttcatctgcaccaccggcaagctgcccgtgccctggcccaccctcgtgaccaccctgacctacggcgtgcagtgcttcagccgctaccccgaccacatgaagcagcacgacttcttcaagtccgccatgcccgaaggctacgtccaggagcgcaccatcttcttcaaggacgacggcaactacaagacccgcgccgaggtgaagttcgagggcgacaccctggtgaaccgcatcgagctgaagggcatcgacttcaaggaggacggcaacatcctgggacacaagctggagtacaactacaacagccacaacgtctatatcatggccgacaagcagaagaacggcatcaaggtgaacttcaagatccgccacaacatcgaggacggcagcgtgcagctcgccgaccactaccagcagaacacccccatcggcgacggccccgtgctgctgcccgacaaccactacctgagcacccagtccgccctgagcaaagaccccaacgagaagcgcgatcacatggtcctgctggagttcgtgaccgccgccgggatcactctcggcatggacgagctgtacaagcaccaccatcaccaccactaacatatgagttatgagatccgaaagtgaaccttgtcctaacccgacagcgaatggcgggagggggcgggctaaaagatcgtattacatagtatttttcccctactctttgtgtttgtcttttttttttttttgaacgcattcaagccacttgtctgggtttacttgtttgtttgcttgcttgcttgcttgcttgcctgcttcttggtcagacggcccaaaaaagggaaaaaattcattcatggcacagataagaaaaagaaaaagtttgtcgaccaccgtcatcagaaagcaagagaagagaaacactcgcgctcacattctcgctcgcgtaagaatcttagccacgcatacgaagtaatttgtccatctggcgaatctttacatgagcgttttcaagctggagcgtgagatcatacctttcttgatcgtaatgttccaaccttgcataggcctcgttgcgatccgctagcaatgcgtcgtactcccgttgcaactgcgccatcgcctcattgtgacgtgagttcagattcttctcgagaccttcgagcgctgctaatttcgcctgacgctccttcttttgtgcttccatgacacgccgcttcaccgtgcgttccacttcttcctcagacatgcccttggctgcctcgacctgctcggtaaaacgggccccagcacgtgctacgagatttcgattccaccgccgccttctatgaaaggttgggcttcggaatcgttttccgggacgccggctggatgatcctccagcgcggggatctcatgctggagttcttcgcccaccccaacttgtttattgcagcttataatggttacaaataaagcaatagcatcacaaatttcacaaataaagcatttttttcactgcattctagttgtggtttgtccaaactcatcaatgtatcttatcatacatggtcgacctgcaggaacctgcattaatgaatcggccaacgcgcggggagaggcggtttgcgtattgggcgctcttccgcttcctcgctcactgactcgctgcgctcggtcgttcggctgcggcgagcggtatcagctcactcaaaggcggtaatacggttatccacagaatcaggggataacgcaggaaagaacatgtgagcaaaaggccagcaaaaggccaggaaccgtaaaaaggccgcgttgctggcgtttttccataggctccgcccccctgacgagcatcacaaaaatcgacgctcaagtcagaggtggcgaaacccgacaggactataaagataccaggcgtttccccctggaagctccctcgtgcgctctcctgttccgaccctgccgcttaccggatacctgtccgcctttctcccttcgggaagcgtggcgctttctcatagctcacgctgtaggtatctcagttcggtgtaggtcgttcgctccaagctgggctgtgtgcacgaaccccccgttcagcccgaccgctgcgccttatccggtaactatcgtcttgagtccaacccggtaagacacgacttatcgccactggcagcagccactggtaacaggattagcagagcgaggtatgtaggcggtgctacagagttcttgaagtggtggcctaactacggctacactagaagaacagtatttggtatctgcgctctgctgaagccagttaccttcggaaaaagagttggtagctcttgatccggcaaacaaaccaccgctggtagcggtggtttttttgtttgcaagcagcagattacgcgcagaaaaaaaggatctcaagaagatcctttgatcttttctacggggtctgacgctcagtggaacgaaaactcacgttaagggattttggtcatgagattatcaaaaaggatcttcacctagatccttttaaattaaaaatgaagttttaaatcaatctaaagtatatatgagtaaacttggtctgacagttaccaatgcttaatcagtgaggcacctatctcagcgatctgtctatttcgttcatccatagttgcctgactccccgtcgtgtagataactacgatacgggagggcttaccatctggccccagtgctgcaatgataccgcgagacccacgctcaccggctccagatttatcagcaataaaccagccagccggaagggccgagcgcagaagtggtcctgcaactttatccgcctccatccagtctattaattgttgccgggaagctagagtaagtagttcgccagttaatagtttgcgcaacgttgttgccattgctacaggcatcgtggtgtcacgctcgtcgtttggtatggcttcattcagctccggttcccaacgatcaaggcgagttacatgatcccccatgttgtgcaaaaaagcggttagctccttcggtcctccgatcgttgtcagaagtaagttggccgcagtgttatcactcatggttatggcagcactgcataattctcttactgtcatgccatccgtaagatgcttttctgtgactggtgagtactcaaccaagtcattctgagaatagtgtatgcggcgaccgagttgctcttgcccggcgtcaatacgggataataccgcgccacatagcagaactttaaaagtgctcatcattggaaaacgttcttcggggcgaaaactctcaaggatcttaccgctgttgagatccagttcgatgtaacccactcgtgcacccaactgatcttcagcatcttttactttcaccagcgtttctgggtgagcaaaaacaggaaggcaaaatgccgcaaaaaagggaataagggcgacacggaaatgttgaatactcatactcttcctttttcaatattattgaagcatttatcagggttattgtctcatgagcggatacatatttgaatgtatttagaaaaataaacaaataggggttccgcgcacatttccccgaaaagtgccacctgacgtctaagaaaccattattatcatgacattaacctataaaaataggcgtatcacgaggccctttcgtctcgcgcgtttcggtgatgacggtgaaaacctctgacacatgcagctcccggagacggtcacagcttgtctgtaagcggatgccgggagcagacaagcccgtcagggcgcgtcagcgggtgttggcgggtgtcggggctggcttaactatgcggcatcagagcagattgtactgagagtgcaccaagcttccaattttaggccccccactgaccgaggtctgtcgataatccacttttccattgattttccaggtttcgttaactcatgccactgagcaaaacttcggtctttcctaacaaaagctctcctcacaaagcatggcgcggcaacggacgtgtcctcatactccactgccacacaaggtcgataaactaagctcctcacaaatagaggagaattccactgacaactgaaaacaatgtatgagagacgatcaccactggagcggcgcggcggttgggcgcggaggtcggcagcaaaaacaagcgactcgccgagcaaacccgaatcagccttcagacggtcgtgcctaacaacacgccgttctaccccgccttcttcgcgccccttcgcgtccaagcatccttcaagtttatctctctagttcaacttcaagaagaacaacaccaccaacaccatgattgaacaagatggattgcacgcaggttctccggccgcttgggtggagaggctattcggctatgactgggcacaacagacaatcggctgctctgatgccgccgtgttccggctgtcagcgcaggggcgcccggttctttttgtcaagaccgacctgtccggtgccctgaatgaactgcaggacgaggcagcgcggctatcgtggctggccacgacgggcgttccttgcgcagctgtgctcgacgttgtcactgaagcgggaagggactggctgctattgggcgaagtgccggggcaggatctcctgtcatctcaccttgctcctgccgagaaagtatccatcatggctgatgcaatgcggcggctgcatacgcttgatccggctacctgcccattcgaccaccaagcgaaacatcgcatcgagcgagcacgtactcggatggaagccggtcttgtcgatcaggatgatctggacgaagagcatcaggggctcgcgccagccgaactgttcgccaggctcaaggcgcgcatgcccgacggcgatgatctcgtcgtgacccatggcgatgcctgcttgccgaatatcatggtggaaaatggccgcttttctggattcatcgactgtggccggctgggtgtggcggaccgctatcaggacatagcgttggctacccgtgatattgctgaagagcttggcggcgaatgggctgaccgcttcctcgtgctttacggtatcgccgctcccgattcgcagcgcatcgccttctatcgccttcttgacgagttcttctgacacgtgctacgagatttcgattccaccgccgccttctatgaaaggttgggcttcggaatcgttttccgggacgccggctggatgatcctccagcgcggggatctcatgctggagttcttcgcccaccccaacttgtttattgcagcttataatggttacaaataaagcaatagcatcacaaatttcacaaataaagcatttttttcactgcattctagttgtggtttgtccaaactcatcaatgtatcttatcatgtctgaattcccggggtac

SEQ ID NO: 92 - DNA, 1314 bp, Artificial
  Codon optimized Isomerase
atggctaaggagtacttcccccagatccagaagattaagttcgagggtaaggacagcaagaacccgctcgcctttcattactacgacgccgagaaggaggtgatgggcaagaagatgaaggactggcttcgctttgctatggcttggtggcacactctctgcgctgagggcgcggaccagtttggcggcggtacgaagagctttccgtggaacgagggcactgacgctattgagattgctaagcagaaggttgacgctggtttcgagattatgcagaagctcggtattccgtactactgctttcacgatgtcgacctcgtttccgagggcaactcgatcgaggagtacgagtcgaacctcaaggctgtggttgcctacctcaaggagaagcagaaggagaccggaatcaagctcctctggagcaccgccaacgttttcggccacaagcgctacatgaacggcgcctccaccaaccctgacttcgatgttgttgcccgcgctattgtccagattaagaacgccatcgacgctggtatcgagctcggagccgagaactacgttttttggggcggacgcgagggttacatgtccctcctcaacaccgaccagaagcgtgagaaggagcacatggccactatgcttaccatggcccgcgactacgcccgcagcaagggttttaagggtacttttctcattgagccgaagcccatggagccgaccaagcaccagtacgacgtcgacaccgagaccgccattggcttccttaaggcccacaaccttgacaaggattttaaggtgaacatcgaggttaaccacgctacgcttgccggccacacctttgagcatgagctcgcctgcgctgttgacgccggaatgcttggttccattgacgccaaccgcggcgactaccagaacggctgggacaccgaccagtttccgattgaccagtacgagctcgtccaggcctggatggagatcatccgtggtggaggctttgttaccggtggtacgaacttcgacgccaagacgcgccgtaacagcacggacctcgaggacatcatcattgctcatgtgtcgggcatggacgccatggctcgcgcccttgagaacgctgctaagctcctccaggagagcccctacacgaagatgaagaaggagcgctacgcgtcgtttgacagcggaatcggtaaggacttcgaggatggcaagctcaccctggagcaggtgtacgagtacggtaagaagaacggcgagccgaagcagaccagcggcaagcaggagctctacgaggccattgtcgccatgtaccagtag

SEQ ID NO: 93 - DNA, 1485 bp, Artificial
  Codon optimized Kinase
atgaagaccgtcgccggcatcgatcttggaacccagtccatgaaggttgtcatttacgactacgagaagaaggagatcatcgagtccgcctcgtgccctatggagctcattagcgagtcggacggaacccgcgagcagacgactgagtggtttgacaagggtctcgaggtgtgctttggaaagctctccgctgataacaagaagaccattgaggcgattggcatctccggccagctccacggcttcgtccctctcgatgcgaacggaaaggcgctctacaacatcaagctctggtgcgacaccgccactgtggaggagtgcaagatcattactgacgccgccggcggcgacaaggctgtcatcgacgcgctcggcaacctcatgctcaccggattcaccgccccgaagattctctggctcaagcgcaacaagcccgaggcctttgctaacctcaagtacattatgctgccccacgattacctcaactggaagctgactggagactacgtcatggagtacggcgacgcctccggcaccgccctttttgattcgaagaaccgctgctggtcgaagaagatttgcgacattattgatcctaagctgctcgaccttctccctaagctcattgagccctcggcccccgccggtaaggtcaacgacgaggccgccaaggcgtacggcattcccgccggaatccccgtttccgctggcggcggtgataacatgatgggtgcggtcggtactggcaccgtcgctgacggattcctcacgatgagcatgggcacctccggaactctttacggctactcggacaagcctatttccgacccggctaacggcctcagcggcttctgcagctccacgggcggctggcttcccctcctttgcaccatgaactgcaccgtcgccaccgagttcgtccgcaacctttttcagatggatatcaaggagctgaacgtcgaggctgctaagtccccctgcggcagcgagggcgttcttgtcattcctttcttcaacggcgagcgcaccccgaacctccccaacggccgcgcctcgattaccggcctcacctccgcgaacacgtcccgcgccaacatcgctcgcgcctcctttgagtcggccgtctttgccatgcgcggtggcctcgatgcgtttcgtaagctcggattccagcccaaggagattcgcctcatcggcggtggttcgaagtccgacctctggcgccagatcgctgctgacattatgaaccttcccatccgtgtcccccttctcgaggaggccgccgccctcggcggagctgtccaggccctttggtgccttaagaaccagtccggtaagtgcgacatcgtcgagctttgcaaggagcatatcaagattgacgagtccaagaacgccaacccgattgccgagaacgtcgccgtgtacgataaggcctacgatgagtactgcaaggtcgttaacacgctcagccctctgtacgcctaa

SEQ ID NO: 94 - DNA, 1569 bp, Artificial
  Codon optimized transporter
atgggcctcgaggataaccgcatggttaagcgctttgtcaacgtgggcgagaagaaggccggtagcaccgccatggccatcattgttggcctcttcgcggcctcgggcggcgtcctcttcggctacgacaccggcactatctcgggcgtcatgactatggactacgttctcgcccgctacccctccaacaagcactccttcaccgctgacgagtcgtcgctcatcgtttccattctttcggtcggcaccttcttcggcgccctctgcgccccgttcctcaacgataccctcggccgccgctggtgcctcatcctcagcgccctcattgtctttaacatcggcgccatcctccaggtcatttccaccgccatccccctgctctgcgcgggccgcgttatcgccggtttcggtgtcggcctcatttccgccaccatcccgctctaccagtccgagactgctccgaagtggattcgcggcgccatcgtttcctgctaccagtgggccatcactatcggacttttcctcgcttcctgcgtcaacaagggcaccgagcacatgaccaactccggttcgtaccgtattcctctggccatccagtgcctctggggcctcatccttggtattggcatgattttcctccctgagaccccccgcttctggatttcgaagggcaaccaggagaaggccgccgagtccctcgcccgtctccgcaagctccccatcgaccatcctgatagccttgaggagcttcgcgatattactgccgcctacgagttcgagaccgtctacggtaagtccagctggtcccaggtcttttcccacaagaaccatcagctcaagcgcctctttaccggcgttgccattcaggcctttcagcagctcaccggagttaactttatcttttactacggcaccaccttttttaagcgcgccggagtcaacggattcaccatcagccttgccaccaacatcgttaacgtcggcagcactattcccggcattcttctcatggaggtcctcggccgccgcaacatgctcatgggcggtgccaccggcatgtcgctgtcgcagcttatcgtcgccattgtcggagttgccacgtcggagaacaacaagtcgagccagtcggtcctcgtcgctttctcgtgcatctttatcgctttttttgccgccacctggggtccctgcgcctgggtcgtcgtcggcgagctctttccccttcgcactcgcgctaagtccgtttccctctgcaccgcgtccaactggctctggaactggggcattgcttacgccaccccctacatggtcgacgaggataagggtaacctcggcagcaacgttttttttatttggggaggcttcaacctcgcttgcgtctttttcgcgtggtacttcatttacgagaccaagggcctttccctcgagcaggttgatgagctctacgagcatgtttcgaaggcgtggaagtccaagggttttgtcccgtccaagcactcctttcgcgagcaggtcgaccagcagatggactccaagaccgaggccattatgagcgaggaggcgtcggtttaa

SEQ ID NO: 95 - DNA, 1512 bp, Artificial
  Codon optimized transporter
atggccctcgaccctgagcagcagcagcccatttcctccgtgtcgcgcgagtttggtaagtcgtccggtgagatctcccccgagcgtgagcctctcattaaggagaaccacgtccccgagaactactccgttgttgccgccatcctccccttcctcttcccggccctgggtggcctcctttacggttacgagattggcgctacgtcgtgcgctacgatttcccttcagtccccctccctctccggcatctcctggtacaacctctcctccgtcgatgttggcctcgtcacttccggttccctctacggtgctctgtttggctccattgttgccttcaccattgccgacgttattggccgtcgcaaggagcttatcctcgctgctctcctctacctcgtcggtgccctcgttaccgctctcgcccctacgtactccgttctcatcatcggccgtgtcatttacggtgtttccgtcggtcttgccatgcatgctgcccctatgtacatcgcggagaccgccccgtcccccatccgcggccagctcgtttccctcaaggagtttttcatcgttctcggtatggtcggcggatacggcattggttccctcaccgtcaacgtccactccggttggcgctacatgtacgctacctccgttcccctcgctgtgatcatgggcattggcatgtggtggcttcctgcctccccccgttggctcctcctccgcgtcattcagggtaagggtaacgttgagaaccagcgcgaggctgccattaagtccctctgctgcctccgtggtcctgccttcgtcgactcggccgccgagcaggtcaacgagattctcgccgagcttaccttcgttggcgaggataaggaggtcaccttcggcgagctcttccagggaaagtgcctcaaggccctcattatcggcggcggccttgttctctttcagcagatcaccggtcagccttcggtcctctactacgccccctcgatcctccagactgcgggcttctccgccgccggcgatgctacccgcgtttccattcttctcggcctcctcaagctcattatgaccggtgtcgccgtcgtcgttatcgatcgtctcggccgtcgccctctcctcctcggcggagtcggtggtatggttgtttcgctctttctccttggctcgtactaccttttcttcagcgcttcccccgtcgtcgccgttgtcgccctccttctctacgtgggttgctaccagctctcctttggccccattggctggcttatgatttccgagatttttcccctcaagctccgtggtcgcggactctcccttgccgtgcttgtcaactttggtgccaacgccctcgtcacctttgccttttcccctctcaaggagctcctcggcgccggcatcctgttttgcggctttggcgttatctgcgttctctcccttgtttttatcttttttatcgtcccggagactaagggcctcacgctcgaggagatcgaggcgaagtgcctctaa

SEQ ID NO: 96 - DNA, 19 bp, Artificial
  Primer 5' CL0130
cctcgggcggcgtcctctt

SEQ ID NO: 97 - DNA, 20 bp, Artificial
  Primer 3' CL0130
ggcggccttctcctggttgc

SEQ ID NO: 98 - DNA, 24 bp, Artificial
  Primer 5' CL0131
ctactccgttgttgccgccatcct

SEQ ID NO: 99 - DNA, 22 bp, Artificial
  Primer 3' CL0131
ccgccgaccataccgagaacga

SEQ ID NO: 100 - DNA, 1362 bp, Artificial
  Codon Optimized NA
atgaaccccaaccagaagattactactatcggtagcatttgcctcgtcgttggacttatctcccttattcttcagattggtaacattatctccatttggatctcgcatagcattcagaccggctcccagaaccacaccggcatttgcaaccagaacattattacttacaagaactccacttgggtcaaggacactactagcgttattcttaccggtaactcgtcgctttgccctattcgcggctgggctatttacagcaaggacaactcgatccgcatcggtagcaagggcgacgtttttgtcatccgtgagccttttatttcctgcagccacctcgagtgccgtactttttttctgactcagggcgctctcctcaacgataagcattccaacggcactgtcaaggatcgcagcccctaccgcgcccttatgtcctgccctgtcggcgaggctcccagcccctacaactcccgttttgagtccgttgcctggtccgccagcgcctgccacgacggaatgggatggctcactattggtatttccggccctgataacggcgctgtcgccgtccttaagtacaacggcattatcaccgagaccatcaagtcctggcgtaagaagatcctccgcacccaggagtccgagtgcgcctgcgtcaacggcagctgcttcacgattatgaccgacggcccctccgacggcctcgcttcctacaagatttttaagattgagaagggtaaggtcacgaagtccatcgagcttaacgccccgaactcccactacgaggagtgctcctgctaccctgacactggcaaggtgatgtgcgtctgccgcgataactggcatggctccaaccgcccctgggttagcttcgatcagaaccttgactaccagattggatacatttgctccggtgtttttggcgacaacccgcgccccgaggatggaactggttcgtgcggtcctgtttacgttgacggcgccaacggcgttaagggtttttcctaccgttacggtaacggagtctggatcggccgcaccaagtcgcacagctcgcgccacggatttgagatgatctgggaccccaacggatggactgagaccgattccaagtttagcgttcgccaggatgtcgttgctatgaccgattggtcgggatactccggttcctttgtgcagcaccctgagctcaccggccttgactgcatgcgcccttgcttttgggtcgagctcattcgcggtcgccctaaggagaagactatttggacctccgccagcagcatttccttttgcggcgttaactccgacaccgtcgactggtcgtggcccgatggcgccgagcttcccttttccattgataag

SEQ ID NO: 101 - DNA, 1431 bp, Artificial
  Codon Optimized NA with V5 tag and a polyhistidine tag
atgaaccccaaccagaagattactactatcggtagcatttgcctcgtcgttggacttatctcccttattcttcagattggtaacattatctccatttggatctcgcatagcattcagaccggctcccagaaccacaccggcatttgcaaccagaacattattacttacaagaactccacttgggtcaaggacactactagcgttattcttaccggtaactcgtcgctttgccctattcgcggctgggctatttacagcaaggacaactcgatccgcatcggtagcaagggcgacgtttttgtcatccgtgagccttttatttcctgcagccacctcgagtgccgtactttttttctgactcagggcgctctcctcaacgataagcattccaacggcactgtcaaggatcgcagcccctaccgcgcccttatgtcctgccctgtcggcgaggctcccagcccctacaactcccgttttgagtccgttgcctggtccgccagcgcctgccacgacggaatgggatggctcactattggtatttccggccctgataacggcgctgtcgccgtccttaagtacaacggcattatcaccgagaccatcaagtcctggcgtaagaagatcctccgcacccaggagtccgagtgcgcctgcgtcaacggcagctgcttcacgattatgaccgacggcccctccgacggcctcgcttcctacaagatttttaagattgagaagggtaaggtcacgaagtccatcgagcttaacgccccgaactcccactacgaggagtgctcctgctaccctgacactggcaaggtgatgtgcgtctgccgcgataactggcatggctccaaccgcccctgggttagcttcgatcagaaccttgactaccagattggatacatttgctccggtgtttttggcgacaacccgcgccccgaggatggaactggttcgtgcggtcctgtttacgttgacggcgccaacggcgttaagggtttttcctaccgttacggtaacggagtctggatcggccgcaccaagtcgcacagctcgcgccacggatttgagatgatctgggaccccaacggatggactgagaccgattccaagtttagcgttcgccaggatgtcgttgctatgaccgattggtcgggatactccggttcctttgtgcagcaccctgagctcaccggccttgactgcatgcgcccttgcttttgggtcgagctcattcgcggtcgccctaaggagaagactatttggacctccgccagcagcatttccttttgcggcgttaactccgacaccgtcgactggtcgtggcccgatggcgccgagcttcccttttccattgataagggtaagcctatccctaaccctctcctcggtctcgattctacgcgtaccggtcatcatcaccatcaccat

SEQ ID NO: 102 - protein, 539 aa, Human parainfluenza 3 virus
MPTSILLIITTMIMASFCQIDITKLQHVGVLVNSPKGMKISQNFETRYLILSLIPKIEDSNSCGDQQIKQYKRLLDRLIIPLYDGLRLQKDVIVSNQESNENTDPRTKRFFGGVIGTIALGVATSAQITAAVALVEAKQARSDIEKLKEAIRDTNKAVQSVQSSIGNLIVAIKSVQDYVNKEIVPSIARLGCEAAGLQLGIALTQHYSELTNIFGDNIGSLQEKGIKLQGIASLYRTNITEIFTTSTVDKYDIYDLLFTESIKVRVIDVDLNDYSITLQVRLPLLTRLLNTQIYRVDSISYNIQNREWYIPLPSHIMTKGAFLGGADVKECIEAFSSYICPSDPGFVLNHEMESCLSGNISQCPRTVVKSDIVPRYAFVNGGVVANCITTTCTCNGIGNRINQPPDQGVKIITHKECNTIGINGMLFNTNKEGTLAFYTPNDITLNNSVALDPIDISIELNKAKSDLEESKEWIRRSNQKLDSIGNWHQSSTTIIIVLIMIIILFIINVTIIIIAVKYYRIQKRNRVDQNDKPYVLTNK

SEQ ID NO: 103 - protein, 511 aa, Vesicular stomatitis Indiana virus
MKCLLYLAFLFIGVNCKFTIVFPHNQKGNWKNVPSNYHYCPSSSDLNWHNDLVGTALQVKMPKSHKAIQADGWMCHASKWVTTCDFRWYGPKYITHSIRSFTPSVEQCKESIEQTKQGTWLNPGFPPQSCGYATVTDAEAAIVQVTPHHVLVDEYTGEWVDSQFINGKCSNDICPTVHNSTTWHSDYKVKGLCDSNLISMDITFFSEDGELSSLGKKGTGFRSNYFAYETGDKACKMQYCKHWGVRLPSGVWFEMADKDLFAAARFPECPEGSSISAPSQTSVDVSLIQDVERILDYSLCQETWSKIRAGLPISPVDLSYLAPKNPGTGPVFTIINGTLKYFETRYIRVDIAAPILSRMVGMISGTTTERVLWDDWAPYEDVGIGPNGVLRTSSGYKFPLYMIGHGMLDSDLHLSSKAQVFEHPHIQDAASQLPDGETLFFGDTGLSKNPIEFVEGWFSSWKSSIASFFFTIGLIIGLFLVLRVGIYLCIKLKHTKKRQIYTDIEMNRLGT